European Patent Application EP 4 344 748 A2, published April 3, 2024. Title: ANTI-GITR ANTIBODIES AND USES THEREOF. Applicant: Regeneron Pharmaceuticals, Inc. Application EP. The sequence listing filed with the application follows.

SEQUENCE LISTING (413 sequences)

SEQ ID NO: 1 - DNA, 369 bp, synthetic construct
  misc_feature 1..369: note = synthetic
  source 1..369: mol_type = other DNA
caggtgcagctggtggagtctgggggaggcgtggtccagcctgggaggtccctgagactctcctgtgcagcgtctggattcaccttcagtagttatggcatggactgggtccgccaggctccaggcaaggggctggagtgggtggcagttatatggtatcctggaagtaataaatactatgcagactccgtgaagggccgattcaccgtctccagagacaattccaagaacacgctgtatctgcaaatgaacagcctgagagccgaggacacggctgtgtattactgtgcgagagacggagaactgggactggactactactccggcatggacgtctggggccaagggaccacggtcaccgtctcctca

SEQ ID NO: 2 - protein, 123 aa, synthetic construct
  REGION 1..123: note = synthetic
QVQLVESGGGVVQPGRSLRLSCAASGFTFSSYGMDWVRQAPGKGLEWVAVIWYPGSNKYYADSVKGRFTVSRDNSKNTLYLQMNSLRAEDTAVYYCARDGELGLDYYSGMDVWGQGTTVTVSS

SEQ ID NO: 3 - DNA, 24 bp, synthetic construct
  misc_feature 1..24: note = synthetic
  source 1..24: mol_type = other DNA
ggattcaccttcagtagttatggc

SEQ ID NO: 4 - protein, 8 aa, synthetic construct
  REGION 1..8: note = synthetic
GFTFSSYG

SEQ ID NO: 5 - DNA, 24 bp, synthetic construct
  misc_feature 1..24: note = synthetic
  source 1..24: mol_type = other DNA
atatggtatcctggaagtaataaa

SEQ ID NO: 6 - protein, 8 aa, synthetic construct
  REGION 1..8: note = synthetic
IWYPGSNK

SEQ ID NO: 7 - DNA, 48 bp, synthetic construct
  misc_feature 1..48: note = synthetic
  source 1..48: mol_type = other DNA
gcgagagacggagaactgggactggactactactccggcatggacgtc

SEQ ID NO: 8 - protein, 16 aa, synthetic construct
  REGION 1..16: note = synthetic
ARDGELGLDYYSGMDV

SEQ ID NO: 9 - DNA, 321 bp, synthetic construct
  misc_feature 1..321: note = synthetic
  source 1..321: mol_type = other DNA
gacatccagatgacccagtctccatcctccctgtctgcatctgtaggagacagagtcaccatcacttgccgggcaagtcagggcattagaaatgatttaaactggtatcagcagaaaccagggaaagcccctaagcgcctgatcaatggtgcatccagtttgcaaagtggggtcccatcaaggttcagcggcagtggatctgggacagaattcactctcacaatcagcagcctgcagcctgaagattttgcaacttattactgtctacaacttaatagttaccctcggacgttcggccaagggaccaaggtggaaatcaaa

SEQ ID NO: 10 - protein, 107 aa, synthetic construct
  REGION 1..107: note = synthetic
DIQMTQSPSSLSASVGDRVTITCRASQGIRNDLNWYQQKPGKAPKRLINGASSLQSGVPSRFSGSGSGTEFTLTISSLQPEDFATYYCLQLNSYPRTFGQGTKVEIK

SEQ ID NO: 11 - DNA, 18 bp, synthetic construct
  misc_feature 1..18: note = synthetic
  source 1..18: mol_type = other DNA
cagggcattagaaatgat

SEQ ID NO: 12 - protein, 6 aa, synthetic construct
  REGION 1..6: note = synthetic
QGIRND

SEQ ID NO: 13-14 - skipped (2 entries)

SEQ ID NO: 15 - DNA, 27 bp, synthetic construct
  misc_feature 1..27: note = synthetic
  source 1..27: mol_type = other DNA
ctacaacttaatagttaccctcggacg

SEQ ID NO: 16 - protein, 9 aa, synthetic construct
  REGION 1..9: note = synthetic
LQLNSYPRT

SEQ ID NO: 17 - DNA, 369 bp, synthetic construct
  misc_feature 1..369: note = synthetic
  source 1..369: mol_type = other DNA
caggtgcagctggtggagtctgggggaggcgtggtccagcctgggaggtccctgagactctcctgtgcagcgtctggattcaccttcagcaactatggcatgcactgggtccgccaggctccaggcaaggggctggagtgggtggcagttatatggtatcctggaagtaataagttctatacagactccgtggagggccgattcaccatctccagagacaattccaagaacacggtatatctacaaatggacagcctgagagccgaagacacggctgtgtattactgtgcgagagggggggcactgggggtagactattactacggtatggacgtctggggccaagggaccacggtcaccgtctcctca

SEQ ID NO: 18 - protein, 123 aa, synthetic construct
  REGION 1..123: note = synthetic
QVQLVESGGGVVQPGRSLRLSCAASGFTFSNYGMHWVRQAPGKGLEWVAVIWYPGSNKFYTDSVEGRFTISRDNSKNTVYLQMDSLRAEDTAVYYCARGGALGVDYYYGMDVWGQGTTVTVSS

SEQ ID NO: 19 - DNA, 24 bp, synthetic construct
  misc_feature 1..24: note = synthetic
  source 1..24: mol_type = other DNA
ggattcaccttcagcaactatggc

SEQ ID NO: 20 - protein, 8 aa, synthetic construct
  REGION 1..8: note = synthetic
GFTFSNYG

SEQ ID NO: 21 - DNA, 24 bp, synthetic construct
  misc_feature 1..24: note = synthetic
  source 1..24: mol_type = other DNA
atatggtatcctggaagtaataag

SEQ ID NO: 22 - protein, 8 aa, synthetic construct
  REGION 1..8: note = synthetic
IWYPGSNK

SEQ ID NO: 23 - DNA, 48 bp, synthetic construct
  misc_feature 1..48: note = synthetic
  source 1..48: mol_type = other DNA
gcgagagggggggcactgggggtagactattactacggtatggacgtc

SEQ ID NO: 24 - protein, 16 aa, synthetic construct
  REGION 1..16: note = synthetic
ARGGALGVDYYYGMDV

SEQ ID NO: 25 - DNA, 321 bp, synthetic construct
  misc_feature 1..321: note = synthetic
  source 1..321: mol_type = other DNA
gccatccagatgacccagtctccatcctccctgtctgcatctgtaggagacagagtcaccctcacttgccgggcaagtcagggcattagaaatgatttaggctggtatcagcagaaaccagggaaagcccctaatttcctgatctattctgcatccagtttacaaagtggggtcccatcaaggttcagcggcagtggatctggcacagatttcactctcaccatcagcagcctacagcctgaggattttgcaacttattactgtctacaaaattacaattacccgtggacgttcggccaagggaccaaggtggaaatcaaa

SEQ ID NO: 26 - protein, 107 aa, synthetic construct
  REGION 1..107: note = synthetic
AIQMTQSPSSLSASVGDRVTLTCRASQGIRNDLGWYQQKPGKAPNFLIYSASSLQSGVPSRFSGSGSGTDFTLTISSLQPEDFATYYCLQNYNYPWTFGQGTKVEIK

SEQ ID NO: 27 - DNA, 18 bp, synthetic construct
  misc_feature 1..18: note = synthetic
  source 1..18: mol_type = other DNA
cagggcattagaaatgat

SEQ ID NO: 28 - protein, 6 aa, synthetic construct
  REGION 1..6: note = synthetic
QGIRND

SEQ ID NO: 29-30 - skipped (2 entries)

SEQ ID NO: 31 - DNA, 27 bp, synthetic construct
  misc_feature 1..27: note = synthetic
  source 1..27: mol_type = other DNA
ctacaaaattacaattacccgtggacg

SEQ ID NO: 32 - protein, 9 aa, synthetic construct
  REGION 1..9: note = synthetic
LQNYNYPWT

SEQ ID NO: 33 - DNA, 372 bp, synthetic construct
  misc_feature 1..372: note = synthetic
  source 1..372: mol_type = other DNA
caggtgcagctggtggagtctgggggaggcgtggtccagcctgggaggtccctgagactctcctgtgttgcgtctggattcaccttcagtgactatggcatgcactgggtccgccaggctccaggcaaggggctagagtgggtggcagttatatggtatgaaggaagtaataaatattatgcagactccgtgacgggccgattcaccatctccagagacaattccaagaacacgctgtttctgcaaatgaacagtctgaaagccgaagacacggctgagtattattgtgcgaaagatggggggcagctcgcctaccagtattactacggcatggacgtctggggccaagggaccacggtcaccgtctcctca

SEQ ID NO: 34 - protein, 124 aa, synthetic construct
  REGION 1..124: note = synthetic
QVQLVESGGGVVQPGRSLRLSCVASGFTFSDYGMHWVRQAPGKGLEWVAVIWYEGSNKYYADSVTGRFTISRDNSKNTLFLQMNSLKAEDTAEYYCAKDGGQLAYQYYYGMDVWGQGTTVTVSS

SEQ ID NO: 35 - DNA, 24 bp, synthetic construct
  misc_feature 1..24: note = synthetic
  source 1..24: mol_type = other DNA
ggattcaccttcagtgactatggc

SEQ ID NO: 36 - protein, 8 aa, synthetic construct
  REGION 1..8: note = synthetic
GFTFSDYG

SEQ ID NO: 37 - DNA, 24 bp, synthetic construct
  misc_feature 1..24: note = synthetic
  source 1..24: mol_type = other DNA
atatggtatgaaggaagtaataaa

SEQ ID NO: 38 - protein, 8 aa, synthetic construct
  REGION 1..8: note = synthetic
IWYEGSNK

SEQ ID NO: 39 - DNA, 51 bp, synthetic construct
  misc_feature 1..51: note = synthetic
  source 1..51: mol_type = other DNA
gcgaaagatggggggcagctcgcctaccagtattactacggcatggacgtc

SEQ ID NO: 40 - protein, 17 aa, synthetic construct
  REGION 1..17: note = synthetic
AKDGGQLAYQYYYGMDV

SEQ ID NO: 41 - DNA, 321 bp, synthetic construct
  misc_feature 1..321: note = synthetic
  source 1..321: mol_type = other DNA
gccatccagatgacccagtctccatcctccctgtctgcatctgtaggagacagagtcaccctcacttgccgggcaagtcagggcattagaaatgatttaggctggtatcagcagaaaccaggaaaagcccctaagagcctgatctatgctgcttccaatttacaaagtggagtcccttcaaggttcagcggcagtggatctggcacagatttcactctcaccatcagcagcctgcagcctgaggattctgcaacttattactgtctacaagactacaattaccctcggacgttcggccaagggaccaaggtggaaatcaaa

SEQ ID NO: 42 - protein, 107 aa, synthetic construct
  REGION 1..107: note = synthetic
AIQMTQSPSSLSASVGDRVTLTCRASQGIRNDLGWYQQKPGKAPKSLIYAASNLQSGVPSRFSGSGSGTDFTLTISSLQPEDSATYYCLQDYNYPRTFGQGTKVEIK

SEQ ID NO: 43 - DNA, 18 bp, synthetic construct
  misc_feature 1..18: note = synthetic
  source 1..18: mol_type = other DNA
cagggcattagaaatgat

SEQ ID NO: 44 - protein, 6 aa, synthetic construct
  REGION 1..6: note = synthetic
QGIRND

SEQ ID NO: 45-46 - skipped (2 entries)

SEQ ID NO: 47 - DNA, 27 bp, synthetic construct
  misc_feature 1..27: note = synthetic
  source 1..27: mol_type = other DNA
ctacaagactacaattaccctcggacg

SEQ ID NO: 48 - protein, 9 aa, synthetic construct
  REGION 1..9: note = synthetic
LQDYNYPRT

SEQ ID NO: 49 - DNA, 369 bp, synthetic construct
  misc_feature 1..369: note = synthetic
  source 1..369: mol_type = other DNA
caggtgcagctggtggagtctgggggaggcgtggtccagcctgggaggtccctgagactctcctgtgcagcgtctggattcaacttcaggagctatggcatgcactgggtccgccaggctccaggcaaggggctggagtgggtggcagttatatggtatgatggaagtaataaatattatgcagactccgtgaagggccgattcaccatctccagagacagttccagggacacgctgtttctgcaaatgaacagcctgagagccggggacacggctgtgtattactgtgcgagaggaggtatgttgggacgggactactactacggtatggacgtctggggccaagggaccacggtcaccgtctcctca

SEQ ID NO: 50 - protein, 123 aa, synthetic construct
  REGION 1..123: note = synthetic
QVQLVESGGGVVQPGRSLRLSCAASGFNFRSYGMHWVRQAPGKGLEWVAVIWYDGSNKYYADSVKGRFTISRDSSRDTLFLQMNSLRAGDTAVYYCARGGMLGRDYYYGMDVWGQGTTVTVSS

SEQ ID NO: 51 - DNA, 24 bp, synthetic construct
  misc_feature 1..24: note = synthetic
  source 1..24: mol_type = other DNA
ggattcaacttcaggagctatggc

SEQ ID NO: 52 - protein, 8 aa, synthetic construct
  REGION 1..8: note = synthetic
GFNFRSYG

SEQ ID NO: 53 - DNA, 24 bp, synthetic construct
  misc_feature 1..24: note = synthetic
  source 1..24: mol_type = other DNA
atatggtatgatggaagtaataaa

SEQ ID NO: 54 - protein, 8 aa, synthetic construct
  REGION 1..8: note = synthetic
IWYDGSNK

SEQ ID NO: 55 - DNA, 48 bp, synthetic construct
  misc_feature 1..48: note = synthetic
  source 1..48: mol_type = other DNA
gcgagaggaggtatgttgggacgggactactactacggtatggacgtc

SEQ ID NO: 56 - protein, 16 aa, synthetic construct
  REGION 1..16: note = synthetic
ARGGMLGRDYYYGMDV

SEQ ID NO: 57 - DNA, 321 bp, synthetic construct
  misc_feature 1..321: note = synthetic
  source 1..321: mol_type = other DNA
gacatccagatgacccagtctccatcctccctgtctgcatctgtaggagacagagtcaccatcacttgccgggcaagtcagggcattagaaatgatttaggctggtatcagcagaaaccagggaaagcccctaagcgcctgatctatgctgcatccagtttgcaaagtggggtcccatcaaggttcagcggcagtggatctgggacagaattcactctcacaatcagcagcctgcagcctgaagattttgcaacttattactgtctacaacataatagttacccgaacacttttggccaggggaccaagctggagatcaaa

SEQ ID NO: 58 - protein, 107 aa, synthetic construct
  REGION 1..107: note = synthetic
DIQMTQSPSSLSASVGDRVTITCRASQGIRNDLGWYQQKPGKAPKRLIYAASSLQSGVPSRFSGSGSGTEFTLTISSLQPEDFATYYCLQHNSYPNTFGQGTKLEIK

SEQ ID NO: 59 - DNA, 18 bp, synthetic construct
  misc_feature 1..18: note = synthetic
  source 1..18: mol_type = other DNA
cagggcattagaaatgat

SEQ ID NO: 60 - protein, 6 aa, synthetic construct
  REGION 1..6: note = synthetic
QGIRND

SEQ ID NO: 61-62 - skipped (2 entries)

SEQ ID NO: 63 - DNA, 27 bp, synthetic construct
  misc_feature 1..27: note = synthetic
  source 1..27: mol_type = other DNA
ctacaacataatagttacccgaacact

SEQ ID NO: 64 - protein, 9 aa, synthetic construct
  REGION 1..9: note = synthetic
LQHNSYPNT

SEQ ID NO: 65 - DNA, 369 bp, synthetic construct
  misc_feature 1..369: note = synthetic
  source 1..369: mol_type = other DNA
caggtgcagctggtggagtctgggggaggcgcggtccagcctgggacgtccctgagactctcctgcgcggcgtctggattcaccttcagtagttttggcatgcactgggtccgccaggctccaggcaaggggctggagtgggtgtcagttatatggtatgaggggagtaataaatattatgcagattcagtgaagggccgattcaccatctccagagacaattccagaaacacgctgagtctgcaaatggacagcctgagagtcgaggacacggctgtgtattactgtgcgagaggtggggaactgggagtcaactactattacgatatggacgtctggggccaagggaccacggtcaccgtctcctca

SEQ ID NO: 66 - protein, 123 aa, synthetic construct
  REGION 1..123: note = synthetic
QVQLVESGGGAVQPGTSLRLSCAASGFTFSSFGMHWVRQAPGKGLEWVSVIWYEGSNKYYADSVKGRFTISRDNSRNTLSLQMDSLRVEDTAVYYCARGGELGVNYYYDMDVWGQGTTVTVSS

SEQ ID NO: 67 - DNA, 24 bp, synthetic construct
  misc_feature 1..24: note = synthetic
  source 1..24: mol_type = other DNA
ggattcaccttcagtagttttggc

SEQ ID NO: 68 - protein, 8 aa, synthetic construct
  REGION 1..8: note = synthetic
GFTFSSFG

SEQ ID NO: 69 - DNA, 24 bp, synthetic construct
  misc_feature 1..24: note = synthetic
  source 1..24: mol_type = other DNA
atatggtatgaggggagtaataaa

SEQ ID NO: 70 - protein, 8 aa, synthetic construct
  REGION 1..8: note = synthetic
IWYEGSNK

SEQ ID NO: 71 - DNA, 48 bp, synthetic construct
  misc_feature 1..48: note = synthetic
  source 1..48: mol_type = other DNA
gcgagaggtggggaactgggagtcaactactattacgatatggacgtc

SEQ ID NO: 72 - protein, 16 aa, synthetic construct
  REGION 1..16: note = synthetic
ARGGELGVNYYYDMDV

SEQ ID NO: 73 - DNA, 321 bp, synthetic construct
  misc_feature 1..321: note = synthetic
  source 1..321: mol_type = other DNA
gacatccagatgacccagtctccatcctccctgtctgcatctgtaggagacagagtcaccatcacttgccgggcaagtcaggacattaaaaatgatttaggctggtttcagcagaaggcaggtaaagcccctaagcgcctgttctatgctacatccagtttgcaaagtggggtcccatcacggttcagcggcagtggatctgggacagaattcactctcacaatcagcagcctgcagcctgaagattttgcaacttattactgtctacaggttcatagttaccctcggacgttcggccaagggaccaaggtggaaatcaaa

SEQ ID NO: 74 - protein, 107 aa, synthetic construct
  REGION 1..107: note = synthetic
DIQMTQSPSSLSASVGDRVTITCRASQDIKNDLGWFQQKAGKAPKRLFYATSSLQSGVPSRFSGSGSGTEFTLTISSLQPEDFATYYCLQVHSYPRTFGQGTKVEIK

SEQ ID NO: 75 - DNA, 18 bp, synthetic construct
  misc_feature 1..18: note = synthetic
  source 1..18: mol_type = other DNA
caggacattaaaaatgat

SEQ ID NO: 76 - protein, 6 aa, synthetic construct
  REGION 1..6: note = synthetic
QDIKND

SEQ ID NO: 77-78 - skipped (2 entries)

SEQ ID NO: 79 - DNA, 27 bp, synthetic construct
  misc_feature 1..27: note = synthetic
  source 1..27: mol_type = other DNA
ctacaggttcatagttaccctcggacg

SEQ ID NO: 80 - protein, 9 aa, synthetic construct
  REGION 1..9: note = synthetic
LQVHSYPRT

SEQ ID NO: 81 - DNA, 369 bp, synthetic construct
  misc_feature 1..369: note = synthetic
  source 1..369: mol_type = other DNA
caggtgcagctggtggagtctgggggaggcgtggtccagcctgggaggtccctgagactctcctgtgaagcgtctggattcaccttcagcaactatggctttcactgggtccgccaggctccaggcaaggggctggattgggtggcagttatatggtatgctggaagtaataagttctatgtagactccgtgcagggccgattcaccatctccagagacaattccaaacaaatattgtttcttcaaatgaacagcctgagagccgaggactcggctgtttattactgtgtgagaggggggatactgggcatagactactactccggtatggacgtctggggccaagggaccacggtcaccgtctcctca

SEQ ID NO: 82 - protein, 123 aa, synthetic construct
  REGION 1..123: note = synthetic
QVQLVESGGGVVQPGRSLRLSCEASGFTFSNYGFHWVRQAPGKGLDWVAVIWYAGSNKFYVDSVQGRFTISRDNSKQILFLQMNSLRAEDSAVYYCVRGGILGIDYYSGMDVWGQGTTVTVSS

SEQ ID NO: 83 - DNA, 24 bp, synthetic construct
  misc_feature 1..24: note = synthetic
  source 1..24: mol_type = other DNA
ggattcaccttcagcaactatggc

SEQ ID NO: 84 - protein, 8 aa, synthetic construct
  REGION 1..8: note = synthetic
GFTFSNYG

SEQ ID NO: 85 - DNA, 24 bp, synthetic construct
  misc_feature 1..24: note = synthetic
  source 1..24: mol_type = other DNA
atatggtatgctggaagtaataag

SEQ ID NO: 86 - protein, 8 aa, synthetic construct
  REGION 1..8: note = synthetic
IWYAGSNK

SEQ ID NO: 87 - DNA, 48 bp, synthetic construct
  misc_feature 1..48: note = synthetic
  source 1..48: mol_type = other DNA
gtgagaggggggatactgggcatagactactactccggtatggacgtc

SEQ ID NO: 88 - protein, 16 aa, synthetic construct
  REGION 1..16: note = synthetic
VRGGILGIDYYSGMDV

SEQ ID NO: 89 - DNA, 321 bp, synthetic construct
  misc_feature 1..321: note = synthetic
  source 1..321: mol_type = other DNA
gccatccagatgacccagtcaccatcctccctgtctgcatctgtaggagacagagtcaccatcacttgccgggcaagtcaggacattagaaatgatttaggctggtatcagcagagaccagggaaggcccctaagttcctgatctattctacatccagtttacaaagtggggtcccatcaagattcagcggcagtggatctggcacagatttcattctcaccatcagcagcctgcagcctgaggattttgccacttattactgtctacaaagtcacaattatccgtggacgttcggccacgggaccaaggtggaaatcaaa

SEQ ID NO: 90 - protein, 107 aa, synthetic construct
  REGION 1..107: note = synthetic
AIQMTQSPSSLSASVGDRVTITCRASQDIRNDLGWYQQRPGKAPKFLIYSTSSLQSGVPSRFSGSGSGTDFILTISSLQPEDFATYYCLQSHNYPWTFGHGTKVEIK

SEQ ID NO: 91 - DNA, 18 bp, synthetic construct
  misc_feature 1..18: note = synthetic
  source 1..18: mol_type = other DNA
caggacattagaaatgat

SEQ ID NO: 92 - protein, 6 aa, synthetic construct
  REGION 1..6: note = synthetic
QDIRND

SEQ ID NO: 93-94 - skipped (2 entries)

SEQ ID NO: 95 - DNA, 27 bp, synthetic construct
  misc_feature 1..27: note = synthetic
  source 1..27: mol_type = other DNA
ctacaaagtcacaattatccgtggacg

SEQ ID NO: 96 - protein, 9 aa, synthetic construct
  REGION 1..9: note = synthetic
LQSHNYPWT

SEQ ID NO: 97 - DNA, 369 bp, synthetic construct
  misc_feature 1..369: note = synthetic
  source 1..369: mol_type = other DNA
caggtgcagctggtggagtctgggggaggcgtggtccagcctgggaggtccctgagactctcctgtgcagtgtctggattcaccctcagtagttatggcatggactgggtccgccaggctccaggcaaggggctggagtgggtggcagttatatggtatgacggaagtaataaatactattcagactccgtgaagggccgattcaccatctccagagacaattccaagaacacactgtttctgcaaatgaacagcctgagagccgacgacacggctgtgtattattgtgcgagagacggggaactgggactggactactactccggtatggacgtctggggccaagggaccacggtcaccgtctcctca

SEQ ID NO: 98 - protein, 123 aa, synthetic construct
  REGION 1..123: note = synthetic
QVQLVESGGGVVQPGRSLRLSCAVSGFTLSSYGMDWVRQAPGKGLEWVAVIWYDGSNKYYSDSVKGRFTISRDNSKNTLFLQMNSLRADDTAVYYCARDGELGLDYYSGMDVWGQGTTVTVSS

SEQ ID NO: 99 - DNA, 24 bp, synthetic construct
  misc_feature 1..24: note = synthetic
  source 1..24: mol_type = other DNA
ggattcaccctcagtagttatggc

SEQ ID NO: 100 - protein, 8 aa, synthetic construct
  REGION 1..8: note = synthetic
GFTLSSYG

SEQ ID NO: 101 - DNA, 24 bp, synthetic construct
  misc_feature 1..24: note = synthetic
  source 1..24: mol_type = other DNA
atatggtatgacggaagtaataaa

SEQ ID NO: 102 - protein, 8 aa, synthetic construct
  REGION 1..8: note = synthetic
IWYDGSNK

SEQ ID NO: 103 - DNA, 48 bp, synthetic construct
  misc_feature 1..48: note = synthetic
  source 1..48: mol_type = other DNA
gcgagagacggggaactgggactggactactactccggtatggacgtc

SEQ ID NO: 104 - protein, 16 aa, synthetic construct
  REGION 1..16: note = synthetic
ARDGELGLDYYSGMDV

SEQ ID NO: 105 - DNA, 321 bp, synthetic construct
  misc_feature 1..321: note = synthetic
  source 1..321: mol_type = other DNA
gacatccagatgacccagtctccatcctccctgtctgcatctgtaggagacagagtcaccatcacttgccgggcaagtcaggacattagaaatgatttaggctggtatcagcagaaaccagggaaagcccctaagcgcctgatctatggtgcatccagtttgcaaagtggtgtcccatcaaggttcagcggcagtggatctgggacagagttcactctcacaatcagcagcctgcagcctgaagattttgcaacttattattgtctacagcttaatagttaccctcggacgttcggccaagggaccaaggtggaaatcaaa

SEQ ID NO: 106 - protein, 107 aa, synthetic construct
  REGION 1..107: note = synthetic
DIQMTQSPSSLSASVGDRVTITCRASQDIRNDLGWYQQKPGKAPKRLIYGASSLQSGVPSRFSGSGSGTEFTLTISSLQPEDFATYYCLQLNSYPRTFGQGTKVEIK

SEQ ID NO: 107 - DNA, 18 bp, synthetic construct
  misc_feature 1..18: note = synthetic
  source 1..18: mol_type = other DNA
caggacattagaaatgat

SEQ ID NO: 108 - protein, 6 aa, synthetic construct
  REGION 1..6: note = synthetic
QDIRND

SEQ ID NO: 109-110 - skipped (2 entries)

SEQ ID NO: 111 - DNA, 27 bp, synthetic construct
  misc_feature 1..27: note = synthetic
  source 1..27: mol_type = other DNA
ctacagcttaatagttaccctcggacg

SEQ ID NO: 112 - protein, 9 aa, synthetic construct
  REGION 1..9: note = synthetic
LQLNSYPRT

SEQ ID NO: 113 - DNA, 354 bp, synthetic construct
  misc_feature 1..354: note = synthetic
  source 1..354: mol_type = other DNA
caggtgcagctggtggagtctgggggaggcgtggtccagcctgggaggtccctgagactctcctgtgcagcctctggattcaccttcagtagctttggcatgcactgggtccgccaggctccaggcaaggggctggagtgggtggcagtgatatcatatgatggaagaaatagatactatgcagactccgtgaagggccgattcaccatctccagagacaattccaagaacacgctgtatctgcaaatgaacagtctgagcgctgaggacacggctatgttttactgtgcgaaagatggctttggcaactcttttgactactggggccagggaaccctggtcaccgtctcctca

SEQ ID NO: 114 - protein, 118 aa, synthetic construct
  REGION 1..118: note = synthetic
QVQLVESGGGVVQPGRSLRLSCAASGFTFSSFGMHWVRQAPGKGLEWVAVISYDGRNRYYADSVKGRFTISRDNSKNTLYLQMNSLSAEDTAMFYCAKDGFGNSFDYWGQGTLVTVSS

SEQ ID NO: 115 - DNA, 24 bp, synthetic construct
  misc_feature 1..24: note = synthetic
  source 1..24: mol_type = other DNA
ggattcaccttcagtagctttggc

SEQ ID NO: 116 - protein, 8 aa, synthetic construct
  REGION 1..8: note = synthetic
GFTFSSFG

SEQ ID NO: 117 - DNA, 24 bp, synthetic construct
  misc_feature 1..24: note = synthetic
  source 1..24: mol_type = other DNA
atatcatatgatggaagaaataga

SEQ ID NO: 118 - protein, 8 aa, synthetic construct
  REGION 1..8: note = synthetic
ISYDGRNR

SEQ ID NO: 119 - DNA, 33 bp, synthetic construct
  misc_feature 1..33: note = synthetic
  source 1..33: mol_type = other DNA
gcgaaagatggctttggcaactcttttgactac

SEQ ID NO: 120 - protein, 11 aa, synthetic construct
  REGION 1..11: note = synthetic
AKDGFGNSFDY

SEQ ID NO: 121 - DNA, 336 bp, synthetic construct
  misc_feature 1..336: note = synthetic
  source 1..336: mol_type = other DNA
gatgttgtgatgactcagtctccactctccctgcccgtcacccttggacagccggcctccatctcctgcaggtctagtcaaagcctcctatacagtgatggaaatacctacttgacttggtttcagcagaggccaggccaatctccaaggcgcctaatttataaggtttctaaccgggactctggggtcccagacagattcagcggcagtgggtcaggcactgatttcacactgacaatcagcagggtggaggctgaggatgttgggatttattactgcatgcaaggcacacactggccgtggacgtttggccaagggaccaaggtggaaatcaaa

SEQ ID NO: 122 - protein, 112 aa, synthetic construct
  REGION 1..112: note = synthetic
DVVMTQSPLSLPVTLGQPASISCRSSQSLLYSDGNTYLTWFQQRPGQSPRRLIYKVSNRDSGVPDRFSGSGSGTDFTLTISRVEAEDVGIYYCMQGTHWPWTFGQGTKVEIK

SEQ ID NO: 123 - DNA, 33 bp, synthetic construct
  misc_feature 1..33: note = synthetic
  source 1..33: mol_type = other DNA
caaagcctcctatacagtgatggaaatacctac

SEQ ID NO: 124 - protein, 11 aa, synthetic construct
  REGION 1..11: note = synthetic
QSLLYSDGNTY

SEQ ID NO: 125-126 - skipped (2 entries)

SEQ ID NO: 127 - DNA, 27 bp, synthetic construct
  misc_feature 1..27: note = synthetic
  source 1..27: mol_type = other DNA
atgcaaggcacacactggccgtggacg

SEQ ID NO: 128 - protein, 9 aa, synthetic construct
  REGION 1..9: note = synthetic
MQGTHWPWT

SEQ ID NO: 129 - DNA, 369 bp, synthetic construct
  misc_feature 1..369: note = synthetic
  source 1..369: mol_type = other DNA
caggtgcagctggtggagtctgggggaggcgtggtccagcctgggaggtccctgagactctcctgtgaagcgtctggattcaccttcagtagctatggcatgcactgggtccgccaggctccaggcaaggggctggagtgggtggcagttatatggtacagtgaaagtaataaatactatacagactccatgaagggccgactcaccatctccagagacaattccaagaacacgctgtatttgcaaatgaacagcctgagagccgaggacacggctgtgtattattgtgcgagaggggggctcctggggaagtactactactacggtatggacgtctggggccaagggaccacggtcaccgtctcctca

SEQ ID NO: 130 - protein, 123 aa, synthetic construct
  REGION 1..123: note = synthetic
QVQLVESGGGVVQPGRSLRLSCEASGFTFSSYGMHWVRQAPGKGLEWVAVIWYSESNKYYTDSMKGRLTISRDNSKNTLYLQMNSLRAEDTAVYYCARGGLLGKYYYYGMDVWGQGTTVTVSS

SEQ ID NO: 131 - DNA, 24 bp, synthetic construct
  misc_feature 1..24: note = synthetic
  source 1..24: mol_type = other DNA
ggattcaccttcagtagctatggc

SEQ ID NO: 132 - protein, 8 aa, synthetic construct
  REGION 1..8: note = synthetic
GFTFSSYG

SEQ ID NO: 133 - DNA, 24 bp, synthetic construct
  misc_feature 1..24: note = synthetic
  source 1..24: mol_type = other DNA
atatggtacagtgaaagtaataaa

SEQ ID NO: 134 - protein, 8 aa, synthetic construct
  REGION 1..8: note = synthetic
IWYSESNK

SEQ ID NO: 135 - DNA, 48 bp, synthetic construct
  misc_feature 1..48: note = synthetic
  source 1..48: mol_type = other DNA
gcgagaggggggctcctggggaagtactactactacggtatggacgtc

SEQ ID NO: 136 - protein, 16 aa, synthetic construct
  REGION 1..16: note = synthetic
ARGGLLGKYYYYGMDV

SEQ ID NO: 137 - DNA, 321 bp, synthetic construct
  misc_feature 1..321: note = synthetic
  source 1..321: mol_type = other DNA
gacatccagatgacccagtctccatcctccctgtctgcatctgtaggagacagagtcattatcacttgccgggcaagtcaggacattagaaatgatttaggctggtatcagcagaaaccagggaaagcccctaagcgcctgatctatgctgcatccagtttgcaaagtggggtcccatcaaggttcagcggcagtggatctgggacagaattcactctcacaatcagcagcctgcagcctgaagattttgcaactttttactgtctacagcttaatagttacccgtacacttttggccaggggaccaagctggagatcaaa

SEQ ID NO: 138 - protein, 107 aa, synthetic construct
  REGION 1..107: note = synthetic
DIQMTQSPSSLSASVGDRVIITCRASQDIRNDLGWYQQKPGKAPKRLIYAASSLQSGVPSRFSGSGSGTEFTLTISSLQPEDFATFYCLQLNSYPYTFGQGTKLEIK

SEQ ID NO: 139 - DNA, 18 bp, synthetic construct
  misc_feature 1..18: note = synthetic
  source 1..18: mol_type = other DNA
caggacattagaaatgat

SEQ ID NO: 140 - protein, 6 aa, synthetic construct
  REGION 1..6: note = synthetic
QDIRND

SEQ ID NO: 141-142 - skipped (2 entries)

SEQ ID NO: 143 - DNA, 27 bp, synthetic construct
  misc_feature 1..27: note = synthetic
  source 1..27: mol_type = other DNA
ctacagcttaatagttacccgtacact

SEQ ID NO: 144 - protein, 9 aa, synthetic construct
  REGION 1..9: note = synthetic
LQLNSYPYT

SEQ ID NO: 145 - DNA, 369 bp, synthetic construct
  misc_feature 1..369: note = synthetic
  source 1..369: mol_type = other DNA
caggtgcagctggtggagtctgggggaggcgtggcccagcctgggaggtccctgagcctctcctgtgcagcgtctggattcaccttcagtgactatggcatgcactgggtccgccaggctccaggcaaggggctggagtgggtggcggttatttggtatgctggaagtaataaatattatgcagactctgtgaaggaccgatttaccatctccagagacaattccaagaacacgctgtatctgcagatgcgcagcctgagagtcgaggacacggctgtatattactgtgcgagagggggggaattgcgtcttgactactactccggtttggacgtctggggccaagggaccacggtcaccgtctcctca

SEQ ID NO: 146 - protein, 123 aa, synthetic construct
  REGION 1..123: note = synthetic
QVQLVESGGGVAQPGRSLSLSCAASGFTFSDYGMHWVRQAPGKGLEWVAVIWYAGSNKYYADSVKDRFTISRDNSKNTLYLQMRSLRVEDTAVYYCARGGELRLDYYSGLDVWGQGTTVTVSS

SEQ ID NO: 147 - DNA, 24 bp, synthetic construct
  misc_feature 1..24: note = synthetic
  source 1..24: mol_type = other DNA
ggattcaccttcagtgactatggc

SEQ ID NO: 148 - protein, 8 aa, synthetic construct
  REGION 1..8: note = synthetic
GFTFSDYG

SEQ ID NO: 149 - DNA, 24 bp, synthetic construct
  misc_feature 1..24: note = synthetic
  source 1..24: mol_type = other DNA
atttggtatgctggaagtaataaa

SEQ ID NO: 150 - protein, 8 aa, synthetic construct
  REGION 1..8: note = synthetic
IWYAGSNK

SEQ ID NO: 151 - DNA, 48 bp, synthetic construct
  misc_feature 1..48: note = synthetic
  source 1..48: mol_type = other DNA
gcgagagggggggaattgcgtcttgactactactccggtttggacgtc

SEQ ID NO: 152 - protein, 16 aa, synthetic construct
  REGION 1..16: note = synthetic
ARGGELRLDYYSGLDV

SEQ ID NO: 153 - DNA, 321 bp, synthetic construct
  misc_feature 1..321: note = synthetic
  source 1..321: mol_type = other DNA
gacatccagatgacccagtctccatcctccctgtctgcatctgtaggagacagagtcaccgtcacttgccgggcaagtcagggcattagaagtgatttaggctggtatcagcagaaaccaggaaaagcccctaagcgcctgatctatgctgcatccagtttccaaagtggggtcccatcaaggttcagcggcagtggatctgggacagaattcactctcacaatcagcagcctgcaccctgaagattttgctacttattactgtctacagtctaataattacccgtggacgttcggccaagggaccaaggtggaaatcaaa

SEQ ID NO: 154 - protein, 107 aa, synthetic construct
  REGION 1..107: note = synthetic
DIQMTQSPSSLSASVGDRVTVTCRASQGIRSDLGWYQQKPGKAPKRLIYAASSFQSGVPSRFSGSGSGTEFTLTISSLHPEDFATYYCLQSNNYPWTFGQGTKVEIK

SEQ ID NO: 155 - DNA, 18 bp, synthetic construct
  misc_feature 1..18: note = synthetic
  source 1..18: mol_type = other DNA
cagggcattagaagtgat

SEQ ID NO: 156 - protein, 6 aa, synthetic construct
  REGION 1..6: note = synthetic
QGIRSD

SEQ ID NO: 157-158 - skipped (2 entries)

SEQ ID NO: 159 - DNA, 27 bp, synthetic construct
  misc_feature 1..27: note = synthetic
  source 1..27: mol_type = other DNA
ctacagtctaataattacccgtggacg

SEQ ID NO: 160 - protein, 9 aa, synthetic construct
  REGION 1..9: note = synthetic
LQSNNYPWT

SEQ ID NO: 161 - DNA, 372 bp, synthetic construct
  misc_feature 1..372: note = synthetic
  source 1..372: mol_type = other DNA
caggtgcagctggtggagtctgggggaggcgtggtccagccgggggggtcccttagactctcctgtgcagtgtctggattcaccttcagtgactatggcatgcactgggtccgccaggttccaggcgcggggctggagtgggtggcagttatttactatgaaggaagtaacaaatactatgcagactccgtgaagggccgattcaccatctccagagacaattccaagaacacgctgtatctgcaaatgaacagcctgagagtcgaggacacgtctatgtatttctgtgcgagaggcccccttctcggcgggaacttctactcttaccttatggacgtctggggccaggggaccacggtcaccgtctcctca

SEQ ID NO: 162 - protein, 124 aa, synthetic construct
  REGION 1..124: note = synthetic
QVQLVESGGGVVQPGGSLRLSCAVSGFTFSDYGMHWVRQVPGAGLEWVAVIYYEGSNKYYADSVKGRFTISRDNSKNTLYLQMNSLRVEDTSMYFCARGPLLGGNFYSYLMDVWGQGTTVTVSS

SEQ ID NO: 163 - DNA, 24 bp, synthetic construct
  misc_feature 1..24: note = synthetic
  source 1..24: mol_type = other DNA
ggattcaccttcagtgactatggc

SEQ ID NO: 164 - protein, 8 aa, synthetic construct
  REGION 1..8: note = synthetic
GFTFSDYG

SEQ ID NO: 165 - DNA, 24 bp, synthetic construct
  misc_feature 1..24: note = synthetic
  source 1..24: mol_type = other DNA
atttactatgaaggaagtaacaaa

SEQ ID NO: 166 - protein, 8 aa, synthetic construct
  REGION 1..8: note = synthetic
IYYEGSNK

SEQ ID NO: 167 - DNA, 51 bp, synthetic construct
  misc_feature 1..51: note = synthetic
  source 1..51: mol_type = other DNA
gcgagaggcccccttctcggcgggaacttctactcttaccttatggacgtc

SEQ ID NO: 168 - protein, 17 aa, synthetic construct
  REGION 1..17: note = synthetic
ARGPLLGGNFYSYLMDV

SEQ ID NO: 169 - DNA, 321 bp, synthetic construct
  misc_feature 1..321: note = synthetic
  source 1..321: mol_type = other DNA
gccatccagatgacccagtctccatcctccctgtctgcatctgtaggagacagagtcaccatcacttgccgggcaagtcagggcattagaaatggtttaggctggtatcagcagaaaccagggaaagcccctaaactcctgatctatactgcatccagtttacaaagtggagtcccatcaagattcagcggcagtggatctggcacagacttcactctcaccatcagcagcctgcagcctgaagattttgcaacttattactgtctacaagattacaattaccctttcagtttcggccctgggaccaaagtggatatcaaa

SEQ ID NO: 170 - protein, 107 aa, synthetic construct
  REGION 1..107: note = synthetic
AIQMTQSPSSLSASVGDRVTITCRASQGIRNGLGWYQQKPGKAPKLLIYTASSLQSGVPSRFSGSGSGTDFTLTISSLQPEDFATYYCLQDYNYPFSFGPGTKVDIK

SEQ ID NO: 171 - DNA, 18 bp, synthetic construct
  misc_feature 1..18: note = synthetic
  source 1..18: mol_type = other DNA
cagggcattagaaatggt

SEQ ID NO: 172 - protein, 6 aa, synthetic construct
  REGION 1..6: note = synthetic
QGIRNG

SEQ ID NO: 173-174 - skipped (2 entries)

SEQ ID NO: 175 - DNA, 27 bp, synthetic construct
  misc_feature 1..27: note = synthetic
  source 1..27: mol_type = other DNA
ctacaagattacaattaccctttcagt

SEQ ID NO: 176 - protein, 9 aa, synthetic construct
  REGION 1..9: note = synthetic
LQDYNYPFS

SEQ ID NO: 177 - DNA, 372 bp, synthetic construct
  misc_feature 1..372: note = synthetic
  source 1..372: mol_type = other DNA
caggtgcagctggtggagtctgggggaggcgtggtccagcctgggaggtccctgagactctcctgtgcagcgtctggatttaccgtcagaaactatggcatgcactgggtccgccaggctccaggcaaggggctggagtgggtggcagttatatggtatgatggaagtaataaatactatgcagactccgtgaagggccgattcaccatctccagagacaattccaagaacacgctgtttctgcaaatgaacagcctgagagccgaggacacggctgtgtattactgtgcgagagggggagagctggtacgtggggactactactacggtatggacgtctggggccaagggaccacggtcaccgtctcctca

SEQ ID NO: 178 - protein, 124 aa, synthetic construct
  REGION 1..124: note = synthetic
QVQLVESGGGVVQPGRSLRLSCAASGFTVRNYGMHWVRQAPGKGLEWVAVIWYDGSNKYYADSVKGRFTISRDNSKNTLFLQMNSLRAEDTAVYYCARGGELVRGDYYYGMDVWGQGTTVTVSS

SEQ ID NO: 179 - DNA, 24 bp, synthetic construct
  misc_feature 1..24: note = synthetic
  source 1..24: mol_type = other DNA
ggatttaccgtcagaaactatggc

SEQ ID NO: 180 - protein, 8 aa, synthetic construct
  REGION 1..8: note = synthetic
GFTVRNYG

SEQ ID NO: 181 - DNA, 24 bp, synthetic construct
  misc_feature 1..24: note = synthetic
  source 1..24: mol_type = other DNA
atatggtatgatggaagtaataaa

SEQ ID NO: 182 - protein, 8 aa, synthetic construct
  REGION 1..8: note = synthetic
IWYDGSNK

SEQ ID NO: 183 - DNA, 51 bp, synthetic construct
  misc_feature 1..51: note = synthetic
  source 1..51: mol_type = other DNA
gcgagagggggagagctggtacgtggggactactactacggtatggacgtc

SEQ ID NO: 184 - protein, 17 aa, synthetic construct
  REGION 1..17: note = synthetic
ARGGELVRGDYYYGMDV

SEQ ID NO: 185 - DNA, 321 bp, synthetic construct
  misc_feature 1..321: note = synthetic
  source 1..321: mol_type = other DNA
gacatccagatgacccagtctccatcctccctgtctgcatctgtaggagacagagtcaccatcacttgccgggcaagtcagggcattagaaatgatttaggctggtatcagcagaaaccagggaaagcccctaagcgcctgatctatggtgcatccagtttgcaaagtggggtcccatcaaggttcagcggcagtggatctgggacagaattcactctcacaatcagcagcctgcagcctgaagattttgcaacttattactgtctacagcataatagttacccgtacacttttggccaggggaccaagctggagatcaaa

SEQ ID NO: 186 - protein, 107 aa, synthetic construct
  REGION 1..107: note = synthetic
DIQMTQSPSSLSASVGDRVTITCRASQGIRNDLGWYQQKPGKAPKRLIYGASSLQSGVPSRFSGSGSGTEFTLTISSLQPEDFATYYCLQHNSYPYTFGQGTKLEIK

SEQ ID NO: 187 - DNA, 18 bp, synthetic construct
  misc_feature 1..18: note = synthetic
  source 1..18: mol_type = other DNA
cagggcattagaaatgat

SEQ ID NO: 188 - protein, 6 aa, synthetic construct
  REGION 1..6: note = synthetic
QGIRND

SEQ ID NO: 189-190 - skipped (2 entries)

SEQ ID NO: 191 - DNA, 27 bp, synthetic construct
  misc_feature 1..27: note = synthetic
  source 1..27: mol_type = other DNA
ctacagcataatagttacccgtacact

SEQ ID NO: 192 - protein, 9 aa, synthetic construct
  REGION 1..9: note = synthetic
LQHNSYPYT

SEQ ID NO: 193 - DNA, 351 bp, synthetic construct
  misc_feature 1..351: note = synthetic
  source 1..351: mol_type = other DNA
caggtgcagctggtggagtctgggggcggcgtggtccagcctgggaggtccctgagactctcctgtgcagcctctggaactatcttcagtacccatggcatgcactgggtccgccaggctccaggcaaggggctggagtgggtggcagttatatcatatgatggaaataagaagtactatgcaggctccgtgaagggccgattcaccatctccagagacaattccaagaacacgctgtatctgcaaatgaacgacgttagatctgaggacacggctgtttatcactgtacgacagatattactggaatcacggactactggggccagggaaccctggtcaccgtctcctca

SEQ ID NO: 194 - protein, 117 aa, synthetic construct
  REGION 1..117: note = synthetic
QVQLVESGGGVVQPGRSLRLSCAASGTIFSTHGMHWVRQAPGKGLEWVAVISYDGNKKYYAGSVKGRFTISRDNSKNTLYLQMNDVRSEDTAVYHCTTDITGITDYWGQGTLVTVSS

SEQ ID NO: 195 - DNA, 24 bp, synthetic construct
  misc_feature 1..24: note = synthetic
  source 1..24: mol_type = other DNA
ggaactatcttcagtacccatggc

SEQ ID NO: 196 - protein, 8 aa, synthetic construct
  REGION 1..8: note = synthetic
GTIFSTHG

SEQ ID NO: 197 - DNA, 24 bp, synthetic construct
  misc_feature 1..24: note = synthetic
  source 1..24: mol_type = other DNA
atatcatatgatggaaataagaag

SEQ ID NO: 198 - protein, 8 aa, synthetic construct
  REGION 1..8: note = synthetic
ISYDGNKK

SEQ ID NO: 199 - DNA, 30 bp, synthetic construct
  misc_feature 1..30: note = synthetic
  source 1..30: mol_type = other DNA
acgacagatattactggaatcacggactac

SEQ ID NO: 200 - protein, 10 aa, synthetic construct
  REGION 1..10: note = synthetic
TTDITGITDY

SEQ ID NO: 201 - DNA, 318 bp, synthetic construct
  misc_feature 1..318: note = synthetic
  source 1..318: mol_type = other DNA
gacatccagatgacccagtctccatcctccctgtctgcatctgtaggagacagagtcaccatcacttgccgggcaagtcagggcattggaaatgatttaggctggtatcagcagaaactagggaaggcccctaagcgcctgatctatgctgcatccagtttggagagtggggtcccatcaaggttcagcggcagtggatccgggacagaattcattctcacaatcagcagcctgcaggctgaagattttgcaacttactactgtctacagcataatggtttcccgacgttcggccaagggaccaaggtggaaatcaaa

SEQ ID NO: 202 - protein, 106 aa, synthetic construct
  REGION 1..106: note = synthetic
DIQMTQSPSSLSASVGDRVTITCRASQGIGNDLGWYQQKLGKAPKRLIYAASSLESGVPSRFSGSGSGTEFILTISSLQAEDFATYYCLQHNGFPTFGQGTKVEIK

SEQ ID NO: 203 - DNA, 18 bp, synthetic construct
  misc_feature 1..18: note = synthetic
  source 1..18: mol_type = other DNA
cagggcattggaaatgat

SEQ ID NO: 204 - protein, 6 aa, synthetic construct
  REGION 1..6: note = synthetic
QGIGND

SEQ ID NO: 205-206 - skipped (2 entries)

SEQ ID NO: 207 - DNA, 24 bp, synthetic construct
  misc_feature 1..24: note = synthetic
  source 1..24: mol_type = other DNA
ctacagcataatggtttcccgacg

SEQ ID NO: 208 - protein, 8 aa, synthetic construct
  REGION 1..8: note = synthetic
LQHNGFPT

SEQ ID NO: 209 - DNA, 363 bp, synthetic construct
  misc_feature 1..363: note = synthetic
  source 1..363: mol_type = other DNA
caggtgcagctggtggagtctgggggaggcgtggtccagcctgggaggtccctgagactctcctgtgcagcgtctggattcaccttcagtaactatggcattcactgggtccgccagcctccaggccagggcctggagtgggtggcagttatatggtatgctggaagtaataagttttatgcagattccgtgaagggccgattcaccatctccagagacaattccaagaactcggcgtatctgcaaatgaacagcctgagagccgaggatacggctgtgtattactgtgcgagagcccccctgggttattactactacggtatggacgtctggggccaagggaccacggtcaccgtctcctca

SEQ ID NO: 210 - protein, 121 aa, synthetic construct
  REGION 1..121: note = synthetic
QVQLVESGGGVVQPGRSLRLSCAASGFTFSNYGIHWVRQPPGQGLEWVAVIWYAGSNKFYADSVKGRFTISRDNSKNSAYLQMNSLRAEDTAVYYCARAPLGYYYYGMDVWGQGTTVTVSS

SEQ ID NO: 211 - DNA, 24 bp, synthetic construct
  misc_feature 1..24: note = synthetic
  source 1..24: mol_type = other DNA
ggattcaccttcagtaactatggc

SEQ ID NO: 212 - protein, 8 aa, synthetic construct
  REGION 1..8: note = synthetic
GFTFSNYG

SEQ ID NO: 213 - DNA, 24 bp, synthetic construct
  misc_feature 1..24: note = synthetic
  source 1..24: mol_type = other DNA
atatggtatgctggaagtaataag

SEQ ID NO: 214 - protein, 8 aa, synthetic construct
  REGION 1..8: note = synthetic
IWYAGSNK

SEQ ID NO: 215 - DNA, 42 bp, synthetic construct
  misc_feature 1..42: note = synthetic
  source 1..42: mol_type = other DNA
gcgagagcccccctgggttattactactacggtatggacgtc

SEQ ID NO: 216 - protein, 14 aa, synthetic construct
  REGION 1..14: note = synthetic
ARAPLGYYYYGMDV

SEQ ID NO: 217 - DNA, 321 bp, synthetic construct
  misc_feature 1..321: note = synthetic
  source 1..321: mol_type = other DNA
gacatccagatgacccagtctccatcctccctgtctgcatctgtaggagacagagtcaccatcacttgccgggcaagtcagggcattagaaatgatttaggctggtatcagcagaaaccagggaaagcccctaagcgcctgatctatgatgcatccagtttggaaagtggggtcccatcaaggttcagcggcagtggatctgggacagaattcactctcacaatcagcagcctgcagcctgaagattttgcaacttattactgtctacagcataatagttacccgtggacgttcggccaagggaccaaggtggaaatcaaa

SEQ ID NO: 218 - protein, 107 aa, synthetic construct
  REGION 1..107: note = synthetic
DIQMTQSPSSLSASVGDRVTITCRASQGIRNDLGWYQQKPGKAPKRLIYDASSLESGVPSRFSGSGSGTEFTLTISSLQPEDFATYYCLQHNSYPWTFGQGTKVEIK

SEQ ID NO: 219 - DNA, 18 bp, synthetic construct
  misc_feature 1..18: note = synthetic
  source 1..18: mol_type = other DNA
cagggcattagaaatgat

SEQ ID NO: 220 - protein, 6 aa, synthetic construct
  REGION 1..6: note = synthetic
QGIRND

SEQ ID NO: 221-222 - skipped (2 entries)

SEQ ID NO: 223 - DNA, 27 bp, synthetic construct
  misc_feature 1..27: note = synthetic
  source 1..27: mol_type = other DNA
ctacagcataatagttacccgtggacg

SEQ ID NO: 224 - protein, 9 aa, synthetic construct
  REGION 1..9: note = synthetic
LQHNSYPWT

SEQ ID NO: 225 - DNA, 375 bp, synthetic construct
  misc_feature 1..375: note = synthetic
  source 1..375: mol_type = other DNA
caggtgcagctggtggagtctgggggaggcgtggtccagcctgggaggtccctgagactctcctgtgcagcgtctggactcaccgtcagtagttatgtcatgcactgggtccgccaggctccaggcaaggggctggagtgggtggcaattatatggtatgatggaagtaataaatactatggagactccgtgaagggccgattcaccatctccagagacaattccaagaaaacgctgtatctgcaaatgaacagcctgagagccgaggacacggctgtgtattactgtgcgagaggccgccccctgtctagtagttcgtccgattattacggtttggacgtctggggccaagggaccacggtcaccgtctcctca

SEQ ID NO: 226 - protein, 125 aa, synthetic construct
  REGION 1..125: note = synthetic
QVQLVESGGGVVQPGRSLRLSCAASGLTVSSYVMHWVRQAPGKGLEWVAIIWYDGSNKYYGDSVKGRFTISRDNSKKTLYLQMNSLRAEDTAVYYCARGRPLSSSSSDYYGLDVWGQGTTVTVSS

SEQ ID NO: 227 - DNA, 24 bp, synthetic construct
  misc_feature 1..24: note = synthetic
  source 1..24: mol_type = other DNA
ggactcaccgtcagtagttatgtc

SEQ ID NO: 228 - protein, 8 aa, synthetic construct
  REGION 1..8: note = synthetic
GLTVSSYV

SEQ ID NO: 229 - DNA, 24 bp, synthetic construct
  misc_feature 1..24: note = synthetic
  source 1..24: mol_type = other DNA
atatggtatgatggaagtaataaa

SEQ ID NO: 230 - protein, 8 aa, synthetic construct
  REGION 1..8: note = synthetic
IWYDGSNK

SEQ ID NO: 231 - DNA, 54 bp, synthetic construct
  misc_feature 1..54: note = synthetic
  source 1..54: mol_type = other DNA
gcgagaggccgccccctgtctagtagttcgtccgattattacggtttggacgtc

SEQ ID NO: 232 - protein, 18 aa, synthetic construct
  REGION 1..18: note = synthetic
ARGRPLSSSSSDYYGLDV

SEQ ID NO: 233 - DNA, 321 bp, synthetic construct
  misc_feature 1..321: note = synthetic
  source 1..321: mol_type = other DNA
gccatccagatgacccagtctccatcctccctgtctgcatctgtaggagacagagtcaccatcatttgccgggcaagtcagggcattagaaatgatttaggctggtatcagcagaaaccagggaaagcccctaacctcctgatctatgctgcatccagtttacaaagtggggtcccatcaaggttcagcggcagtggatctggcacagatttcactctcaccatcagcagcctgcagcctgaagattttgcaacttattactgtctacaagattacaattatccgtggacgttcggccaagggaccaaggtggaaatcaaa

SEQ ID NO: 234 - protein, 107 aa, synthetic construct
  REGION 1..107: note = synthetic
AIQMTQSPSSLSASVGDRVTIICRASQGIRNDLGWYQQKPGKAPNLLIYAASSLQSGVPSRFSGSGSGTDFTLTISSLQPEDFATYYCLQDYNYPWTFGQGTKVEIK

SEQ ID NO: 235 - DNA, 18 bp, synthetic construct
  misc_feature 1..18: note = synthetic
  source 1..18: mol_type = other DNA
cagggcattagaaatgat

SEQ ID NO: 236 - protein, 6 aa, synthetic construct
  REGION 1..6: note = synthetic
QGIRND

SEQ ID NO: 237-238 - skipped (2 entries)

SEQ ID NO: 239 - DNA, 27 bp, synthetic construct
  misc_feature 1..27: note = synthetic
  source 1..27: mol_type = other DNA
ctacaagattacaattatccgtggacg

SEQ ID NO: 240 - protein, 9 aa, synthetic construct
  REGION 1..9: note = synthetic
LQDYNYPWT

SEQ ID NO: 241 - DNA, 360 bp, synthetic construct
  misc_feature 1..360: note = synthetic
  source 1..360: mol_type = other DNA
gaggtgcagctggtggagtctgggggaggcctggtacagcctggagggtccctgagactctcctgtgcagcctctggattcaccttcagtaattatgaaatgtattgggtccgccaggctccagggaaggggctggaatgggtttcatacattagtagtagtggtactaccatatactacgcagactctgtgaagggccgattcagtgtctccagagaaaacgccaggagctcactgtatctgcaaatgaacagtctgagagtcgaggactcggctgtttacttctgtgcgaagtataactggaactccttctatggtttggacgtctggggccaagggaccacggtcaccgtctcctca

SEQ ID NO: 242 - protein, 120 aa, synthetic construct
  REGION 1..120: note = synthetic
EVQLVESGGGLVQPGGSLRLSCAASGFTFSNYEMYWVRQAPGKGLEWVSYISSSGTTIYYADSVKGRFSVSRENARSSLYLQMNSLRVEDSAVYFCAKYNWNSFYGLDVWGQGTTVTVSS

SEQ ID NO: 243 - DNA, 24 bp, synthetic construct
  misc_feature 1..24: note = synthetic
  source 1..24: mol_type = other DNA
ggattcaccttcagtaattatgaa

SEQ ID NO: 244 - protein, 8 aa, synthetic construct
  REGION 1..8: note = synthetic
GFTFSNYE

SEQ ID NO: 245 - DNA, 24 bp, synthetic construct
  misc_feature 1..24: note = synthetic
  source 1..24: mol_type = other DNA
attagtagtagtggtactaccata

SEQ ID NO: 246 - protein, 8 aa, synthetic construct
  REGION 1..8: note = synthetic
ISSSGTTI

SEQ ID NO: 247 - DNA, 39 bp, synthetic construct
  misc_feature 1..39: note = synthetic
  source 1..39: mol_type = other DNA
gcgaagtataactggaactccttctatggtttggacgtc

SEQ ID NO: 248 - protein, 13 aa, synthetic construct
  REGION 1..13: note = synthetic
AKYNWNSFYGLDV

SEQ ID NO: 249 - DNA, 321 bp, synthetic construct
  misc_feature 1..321: note = synthetic
  source 1..321: mol_type = other DNA
gccatccagatgacccagtctccatcctccctgtctgcatctgtaggagacagagtcaccatcacttgccgggcaagtcaggacattagaaatgatttaggctggtatcagcagaaaccagggaaagcccctaagctcctgatctctgctgcatccagtttacagggtggggtcccatcaaggttcagcggcagtggatctggcacagatttcactctcaccattagcagcctgcagcctgcagattttgcaacttattactgtctacaagagtacaattatgcactcactttcggcggagggaccaaggtggagatcaaa

SEQ ID NO: 250 - protein, 107 aa, synthetic construct
  REGION 1..107: note = synthetic
AIQMTQSPSSLSASVGDRVTITCRASQDIRNDLGWYQQKPGKAPKLLISAASSLQGGVPSRFSGSGSGTDFTLTISSLQPADFATYYCLQEYNYALTFGGGTKVEIK

SEQ ID NO: 251 - DNA, 18 bp, synthetic construct
  misc_feature 1..18: note = synthetic
  source 1..18: mol_type = other DNA
caggacattagaaatgat

SEQ ID NO: 252 - protein, 6 aa, synthetic construct
  REGION 1..6: note = synthetic
QDIRND

SEQ ID NO: 253-254 - skipped (2 entries)

SEQ ID NO: 255 - DNA, 27 bp, synthetic construct
  misc_feature 1..27: note = synthetic
  source 1..27: mol_type = other DNA
ctacaagagtacaattatgcactcact

SEQ ID NO: 256 - protein, 9 aa, synthetic construct
  REGION 1..9: note = synthetic
LQEYNYALT

SEQ ID NO: 257 - DNA, 369 bp, synthetic construct
  misc_feature 1..369: note = synthetic
  source 1..369: mol_type = other DNA
gaggtgcagctggtggagtctgggggaggtttggtccagcctggagggtccctgagactctcctgtgcagcctctggattcaccttcagggtttatgaaatgaactgggtccgccaggctccagggaaggggctggagtggatttcatacattggcagtagtggttttaccatatactacgcagactctgtgaagggccgattcaccatctccagagacaacgccaagaactcactgtttctgcagctgaacagcctgagagccgaggacacggctgtttattactgtgcgagagggtggaacgacggagttcctaactatttgggtatggacgtctggggccaaggcaccacggtcaccgtctcctca

SEQ ID NO: 258 - protein, 123 aa, synthetic construct
  REGION 1..123: note = synthetic
EVQLVESGGGLVQPGGSLRLSCAASGFTFRVYEMNWVRQAPGKGLEWISYIGSSGFTIYYADSVKGRFTISRDNAKNSLFLQLNSLRAEDTAVYYCARGWNDGVPNYLGMDVWGQGTTVTVSS

SEQ ID NO: 259 - DNA, 24 bp, synthetic construct
  misc_feature 1..24: note = synthetic
  source 1..24: mol_type = other DNA
ggattcaccttcagggtttatgaa

SEQ ID NO: 260 - protein, 8 aa, synthetic construct
  REGION 1..8: note = synthetic
GFTFRVYE

SEQ ID NO: 261 - DNA, 24 bp, synthetic construct
  misc_feature 1..24: note = synthetic
  source 1..24: mol_type = other DNA
attggcagtagtggttttaccata

SEQ ID NO: 262 - protein, 8 aa, synthetic construct
  REGION 1..8: note = synthetic
IGSSGFTI

SEQ ID NO: 263 - DNA, 48 bp, synthetic construct
  misc_feature 1..48: note = synthetic
  source 1..48: mol_type = other DNA
gcgagagggtggaacgacggagttcctaactatttgggtatggacgtc

SEQ ID NO: 264 - protein, 16 aa, synthetic construct
  REGION 1..16: note = synthetic
ARGWNDGVPNYLGMDV

SEQ ID NO: 265 - DNA, 321 bp, synthetic construct
  misc_feature 1..321: note = synthetic
  source 1..321: mol_type = other DNA
gacatccagatgacccagtctccatcctccctgtctgcatctgtaggagacagagtcaccatcacttgccaggcgagtcaggacattaacaaatatttaaattggtatcagcagaaaccaggaaaagcccctaaactcctgatctacgatgcatccaatttggaaacaggggtcccatcaaggttcagtggaagtggatctgggacagattttactttcaccatcagcagcctgcagcctgaagatattgcaagatatcactgtcaacagtatgataaaatcccgctcactttcggcggagggaccaaggtggagatcaaa

SEQ ID NO: 266 - protein, 107 aa, synthetic construct
  REGION 1..107: note = synthetic
DIQMTQSPSSLSASVGDRVTITCQASQDINKYLNWYQQKPGKAPKLLIYDASNLETGVPSRFSGSGSGTDFTFTISSLQPEDIARYHCQQYDKIPLTFGGGTKVEIK

SEQ ID NO: 267 - DNA, 18 bp, synthetic construct
  misc_feature 1..18: note = synthetic
  source 1..18: mol_type = other DNA
caggacattaacaaatat

SEQ ID NO: 268 - protein, 6 aa, synthetic construct
  REGION 1..6: note = synthetic
QDINKY

SEQ ID NO: 269-270 - skipped (2 entries)

SEQ ID NO: 271 - DNA, 27 bp, synthetic construct
  misc_feature 1..27: note = synthetic
  source 1..27: mol_type = other DNA
caacagtatgataaaatcccgctcact

SEQ ID NO: 272 - protein, 9 aa, synthetic construct
  REGION 1..9: note = synthetic
QQYDKIPLT

SEQ ID NO: 273 - DNA, 369 bp, synthetic construct
  misc_feature 1..369: note = synthetic
  source 1..369: mol_type = other DNA
caggtgcagctggtggagtctgggggaggcgtggtccagcctgggaggtccctgagactctcctgtgcagcgtctggattcaccttcagcagctatggcatgcactgggtccgccaggctccaggcaaggggctggagtgggtggcagttatctggtatgttggaagtaataaatactatggagagtccgtgaagggccgattcaccatctccagagacaattccaagaacacgctgtatttgcaaatgaacagcctgagagacgaggacacggctatatattactgtgcgagagggggtcaactgggctccttctactattacggtatggacgtctggggccaagggaccacggtcaccgtctcctca

SEQ ID NO: 274 - protein, 123 aa, synthetic construct
  REGION 1..123: note = synthetic
QVQLVESGGGVVQPGRSLRLSCAASGFTFSSYGMHWVRQAPGKGLEWVAVIWYVGSNKYYGESVKGRFTISRDNSKNTLYLQMNSLRDEDTAIYYCARGGQLGSFYYYGMDVWGQGTTVTVSS

SEQ ID NO: 275 - DNA, 24 bp, synthetic construct
  misc_feature 1..24: note = synthetic
  source 1..24: mol_type = other DNA
ggattcaccttcagcagctatggc

SEQ ID NO: 276 - protein, 8 aa, synthetic construct
  REGION 1..8: note = synthetic
GFTFSSYG

SEQ ID NO: 277 - DNA, 24 bp, synthetic construct
  misc_feature 1..24: note = synthetic
  source 1..24: mol_type = other DNA
atctggtatgttggaagtaataaa

SEQ ID NO: 278 - protein, 8 aa, synthetic construct
  REGION 1..8: note = synthetic
IWYVGSNK

SEQ ID NO: 279 - DNA, 48 bp, synthetic construct
  misc_feature 1..48: note = synthetic
  source 1..48: mol_type = other DNA
gcgagagggggtcaactgggctccttctactattacggtatggacgtc

SEQ ID NO: 280 - protein, 16 aa, synthetic construct
  REGION 1..16: note = synthetic
ARGGQLGSFYYYGMDV

SEQ ID NO: 281 - DNA, 321 bp, synthetic construct
  misc_feature 1..321: note = synthetic
  source 1..321: mol_type = other DNA
gacatccagatgacccagtctccatcctccctgtctgcatctgtaggagacagagtcaccatcacttgccgggcaagtcagggcattagaaatgatttaggctggtatcagcagaaaccagggaaagcccctaagcgcctgatctatgatgtatccagtttacaaagtggggtcccatcaaggttcagcggcagtggatctgggacagaattcactctcacaatcagcagcctgcagcctgaagatcttgcaacttattactgtctacagcataatagttacccgtggacgttcggccaagggaccaaggtggaaatcaaa

SEQ ID NO: 282 - protein, 107 aa, synthetic construct
  REGION 1..107: note = synthetic
DIQMTQSPSSLSASVGDRVTITCRASQGIRNDLGWYQQKPGKAPKRLIYDVSSLQSGVPSRFSGSGSGTEFTLTISSLQPEDLATYYCLQHNSYPWTFGQGTKVEIK

SEQ ID NO: 283 - DNA, 18 bp, synthetic construct
  misc_feature 1..18: note = synthetic
  source 1..18: mol_type = other DNA
cagggcattagaaatgat

SEQ ID NO: 284 - protein, 6 aa, synthetic construct
  REGION 1..6: note = synthetic
QGIRND

SEQ ID NO: 285-286 - skipped (2 entries)

SEQ ID NO: 287 - DNA, 27 bp, synthetic construct
  misc_feature 1..27: note = synthetic
  source 1..27: mol_type = other DNA
ctacagcataatagttacccgtggacg

SEQ ID NO: 288 - protein, 9 aa, synthetic construct
  REGION 1..9: note = synthetic
LQHNSYPWT

SEQ ID NO: 289 - DNA, 360 bp, synthetic construct
  misc_feature 1..360: note = synthetic
  source 1..360: mol_type = other DNA
caggtgcagctggtggagtctgggggaggcgtggtccagcctgggaggtccctgagaatttcctgtgcagcgtcaggattcaccttcaataactatggcttccactgggtccgccaggctccaggcagggggctggagtgggtggcagttatttggtattctggaagtaataaatactatggagactccgtgaagggccgattcaccatctccagagacaattccaaaaatatattgtatctgcaaatgaacagtctgagagccgaggacacggctatatattactgtgcgagatttccgtttagcagcagttggctcttggactactggggccagggaaccctggtcaccgtctcctca

SEQ ID NO: 290 - protein, 120 aa, synthetic construct
  REGION 1..120: note = synthetic
QVQLVESGGGVVQPGRSLRISCAASGFTFNNYGFHWVRQAPGRGLEWVAVIWYSGSNKYYGDSVKGRFTISRDNSKNILYLQMNSLRAEDTAIYYCARFPFSSSWLLDYWGQGTLVTVSS

SEQ ID NO: 291 - DNA, 24 bp, synthetic construct
  misc_feature 1..24: note = synthetic
  source 1..24: mol_type = other DNA
ggattcaccttcaataactatggc

SEQ ID NO: 292 - protein, 8 aa, synthetic construct
  REGION 1..8: note = synthetic
GFTFNNYG

SEQ ID NO: 293 - DNA, 24 bp, synthetic construct
  misc_feature 1..24: note = synthetic
  source 1..24: mol_type = other DNA
atttggtattctggaagtaataaa

SEQ ID NO: 294 - protein, 8 aa, synthetic construct
  REGION 1..8: note = synthetic
IWYSGSNK

SEQ ID NO: 295 - DNA, 39 bp, synthetic construct
  misc_feature 1..39: note = synthetic
  source 1..39: mol_type = other DNA
gcgagatttccgtttagcagcagttggctcttggactac

SEQ ID NO: 296 - protein, 13 aa, synthetic construct
  REGION 1..13: note = synthetic
ARFPFSSSWLLDY

SEQ ID NO: 297 - DNA, 321 bp, synthetic construct
  misc_feature 1..321: note = synthetic
  source 1..321: mol_type = other DNA
gacatccagttgacccagtctccatccttcctgtctgcatctgtaggagacagagtcaccttcacttgctgggccagtcagggcattagtgattatttagcctggtatcaacaaaaaccagggaaagcccctaaactcctgatctatgctgcatccgctttgcaaagtggggtcccatcaaggttcagcggcagtggatctgggacagaattcactctcacagtcagcagcctacagcctgaagattttgcaacttattactgtcaacagcttaatagttatccattcactttcggccctgggaccaaagtggatatcaaa

SEQ ID NO: 298 - protein, 107 aa, synthetic construct
  REGION 1..107: note = synthetic
DIQLTQSPSFLSASVGDRVTFTCWASQGISDYLAWYQQKPGKAPKLLIYAASALQSGVPSRFSGSGSGTEFTLTVSSLQPEDFATYYCQQLNSYPFTFGPGTKVDIK

SEQ ID NO: 299 - DNA, 18 bp, synthetic construct
  misc_feature 1..18: note = synthetic
  source 1..18: mol_type = other DNA
cagggcattagtgattat

SEQ ID NO: 300 - protein, 6 aa, synthetic construct
  REGION 1..6: note = synthetic
QGISDY

SEQ ID NO: 301-302 - skipped (2 entries)

SEQ ID NO: 303 - DNA, 27 bp, synthetic construct
  misc_feature 1..27: note = synthetic
  source 1..27: mol_type = other DNA
caacagcttaatagttatccattcact

SEQ ID NO: 304 - protein, 9 aa, synthetic construct
  REGION 1..9: note = synthetic
QQLNSYPFT

SEQ ID NO: 305 - DNA, 357 bp, synthetic construct
  misc_feature 1..357: note = synthetic
  source 1..357: mol_type = other DNA
cagctgcagctgcaggagtcgggcccaggactggtgaagccttcggagaccctgtccctcacctgcactgtctctggtggctccatcagcagtactaatcactactggggctggatccgccagcccccagggaagggcctggagtggatcggtaatgtctattatattgggaacgcctactacaacccgtccctcaagactggagtcaccttttccgtagacacgtccaagaaccagttctccctgaacctgaggtctgtgaccgccgcagacacggctatgtattactgtgcgagactttctaactggaatttcttggacttgtggggccagggaaccctggtcaccgtctcctca

SEQ ID NO: 306 - protein, 119 aa, synthetic construct
  REGION 1..119: note = synthetic
QLQLQESGPGLVKPSETLSLTCTVSGGSISSTNHYWGWIRQPPGKGLEWIGNVYYIGNAYYNPSLKTGVTFSVDTSKNQFSLNLRSVTAADTAMYYCARLSNWNFLDLWGQGTLVTVSS

SEQ ID NO: 307 - DNA, 30 bp, synthetic construct
  misc_feature 1..30: note = synthetic
  source 1..30: mol_type = other DNA
ggtggctccatcagcagtactaatcactac

SEQ ID NO: 308 - protein, 10 aa, synthetic construct
  REGION 1..10: note = synthetic
GGSISSTNHY

SEQ ID NO: 309 - DNA, 21 bp, synthetic construct
  misc_feature 1..21: note = synthetic
  source 1..21: mol_type = other DNA
gtctattatattgggaacgcc

SEQ ID NO: 310 - protein, 7 aa, synthetic construct
  REGION 1..7: note = synthetic
VYYIGNA

SEQ ID NO: 311 - DNA, 33 bp, synthetic construct
  misc_feature 1..33: note = synthetic
  source 1..33: mol_type = other DNA
gcgagactttctaactggaatttcttggacttg

SEQ ID NO: 312 - protein, 11 aa, synthetic construct
  REGION 1..11: note = synthetic
ARLSNWNFLDL

SEQ ID NO: 313 - DNA, 318 bp, synthetic construct
  misc_feature 1..318: note = synthetic
  source 1..318: mol_type = other DNA
gaaattgtgatgacgcagtctccagccaccctgtctgtgtctccaggggaaagagccaccctctcctgcagggccagtcagagtattagcagcaacttagcctggtaccagcagaaacctggccaggctcccaggctcctcatctatggtgcatccaccagggccactggtatcccagccaggttcagtggcagtgggtctgggacagagttcactctcaccatcagcagcctgcagtctgaagattttgcagtttattactgtcagcaatttaataactggctctctttcggcggagggaccaaggtggagatcaaa

SEQ ID NO: 314 - protein, 106 aa, synthetic construct
  REGION 1..106: note = synthetic
EIVMTQSPATLSVSPGERATLSCRASQSISSNLAWYQQKPGQAPRLLIYGASTRATGIPARFSGSGSGTEFTLTISSLQSEDFAVYYCQQFNNWLSFGGGTKVEIK

SEQ ID NO: 315 - DNA, 18 bp, synthetic construct
  misc_feature 1..18: note = synthetic
  source 1..18: mol_type = other DNA
cagagtattagcagcaac

SEQ ID NO: 316 - protein, 6 aa, synthetic construct
  REGION 1..6: note = synthetic
QSISSN

SEQ ID NO: 317-318 - skipped (2 entries)

SEQ ID NO: 319 - DNA, 24 bp, synthetic construct
  misc_feature 1..24: note = synthetic
  source 1..24: mol_type = other DNA
cagcaatttaataactggctctct

SEQ ID NO: 320 - protein, 8 aa, synthetic construct
  REGION 1..8: note = synthetic
QQFNNWLS

SEQ ID NO: 321 - DNA, 366 bp, synthetic construct
  misc_feature 1..366: note = synthetic
  source 1..366: mol_type = other DNA
caggtgcagctggtggagtcgggggggggcgtggtccagcctgggaggtccctgagactctcctgtgcagcgtctggattcaccttcagtacctatggcatgcactgggtccgccaggctccaggcaaggggctggagtgggtggcagttatatggtatgttggaagtaataaattctatgcagactccgtgaagggccgattcaccatctccagagacaattccaagaacacgctgtatctgcaaatggacagcctgagagccgaggacacgggtgtgtatcactgtgcgagagacagtatggttcggccctattattacggtatggacgtctggggccaagggaccacggtcaccgtctcctca

SEQ ID NO: 322 - protein, 122 aa, synthetic construct
  REGION 1..122: note = synthetic
QVQLVESGGGVVQPGRSLRLSCAASGFTFSTYGMHWVRQAPGKGLEWVAVIWYVGSNKFYADSVKGRFTISRDNSKNTLYLQMDSLRAEDTGVYHCARDSMVRPYYYGMDVWGQGTTVTVSS

SEQ ID NO: 323 - DNA, 24 bp, synthetic construct
  misc_feature 1..24: note = synthetic
  source 1..24: mol_type = other DNA
ggattcaccttcagtacctatggc

SEQ ID NO: 324 - protein, 8 aa, synthetic construct
  REGION 1..8: note = synthetic
GFTFSTYG

SEQ ID NO: 325 - DNA, 24 bp, synthetic construct
  misc_feature 1..24: note = synthetic
  source 1..24: mol_type = other DNA
atatggtatgttggaagtaataaa

SEQ ID NO: 326 - protein, 8 aa, synthetic construct
  REGION 1..8: note = synthetic
IWYVGSNK

SEQ ID NO: 327 - DNA, 45 bp, synthetic construct
  misc_feature 1..45: note = synthetic
  source 1..45: mol_type = other DNA
gcgagagacagtatggttcggccctattattacggtatggacgtc

SEQ ID NO: 328 - protein, 15 aa, synthetic construct
  REGION 1..15: note = synthetic
ARDSMVRPYYYGMDV

SEQ ID NO: 329 - DNA, 375 bp, synthetic construct
  misc_feature 1..375: note = synthetic
  source 1..375: mol_type = other DNA
caggtgcagctggtggagtctgggggaggcgtggtccaacctgggaggtccctgagactctcctgttcagcgtctggattcaccctcagtaattttgtcatgcattgggtccgccaggctccaggcaaggggctggagtgggtggcagtcatattatatgatggaagtaataaatattatgcggactccgtgaagggccgattcaccatctccagagacaattccaacaacaggctgtatctgcaaatgaacagcctgagagccgaggacacggctctttattactgtgcgagaggagagtccttgggatcacctatctattattactacggtttggacgtctggggccaagggaccacggtcaccgtctcctca

SEQ ID NO: 330 - protein, 125 aa, synthetic construct
  REGION 1..125: note = synthetic
QVQLVESGGGVVQPGRSLRLSCSASGFTLSNFVMHWVRQAPGKGLEWVAVILYDGSNKYYADSVKGRFTISRDNSNNRLYLQMNSLRAEDTALYYCARGESLGSPIYYYYGLDVWGQGTTVTVSS

SEQ ID NO: 331 - DNA, 24 bp, synthetic construct
  misc_feature 1..24: note = synthetic
  source 1..24: mol_type = other DNA
ggattcaccctcagtaattttgtc

SEQ ID NO: 332 - protein, 8 aa, synthetic construct
  REGION 1..8: note = synthetic
GFTLSNFV

SEQ ID NO: 333 - DNA, 24 bp, synthetic construct
  misc_feature 1..24: note = synthetic
  source 1..24: mol_type = other DNA
atattatatgatggaagtaataaa

SEQ ID NO: 334 - protein, 8 aa, synthetic construct
  REGION 1..8: note = synthetic
ILYDGSNK

SEQ ID NO: 335 - DNA, 54 bp, synthetic construct
  misc_feature 1..54: note = synthetic
  source 1..54: mol_type = other DNA
gcgagaggagagtccttgggatcacctatctattattactacggtttggacgtc

SEQ ID NO: 336 - protein, 18 aa, synthetic construct
  REGION 1..18: note = synthetic
ARGESLGSPIYYYYGLDV

SEQ ID NO: 337 - DNA, 360 bp, synthetic construct
  misc_feature 1..360: note = synthetic
  source 1..360: mol_type = other DNA
caggtgcagctgcaggagtcgggcccaggactggtgaagccttcggagaccctgtccctcacctgcattgtctctggtggctccatcagtggttacttctggaactggatccggcagcccccagggaagggacttgaatggattggttatatctattacagtgggaccaccatctacaacccctccctcaagagtcgattcaccatatcactagacacgtccaagaaccagttctccctaaagctgacctctgtgaccgctgcggacacggccgtatattactgtgcgagagagtcgtataatccctcgccgcgatattttgaccactggggccagggaaccctggtcaccgtctcctca

SEQ ID NO: 338 - protein, 120 aa, synthetic construct
  REGION 1..120: note = synthetic
QVQLQESGPGLVKPSETLSLTCIVSGGSISGYFWNWIRQPPGKGLEWIGYIYYSGTTIYNPSLKSRFTISLDTSKNQFSLKLTSVTAADTAVYYCARESYNPSPRYFDHWGQGTLVTVSS

SEQ ID NO: 339 - DNA, 24 bp, synthetic construct
  misc_feature 1..24: note = synthetic
  source 1..24: mol_type = other DNA
ggtggctccatcagtggttacttc

SEQ ID NO: 340 - protein, 8 aa, synthetic construct
  REGION 1..8: note = synthetic
GGSISGYF

SEQ ID NO: 341 - DNA, 21 bp, synthetic construct
  misc_feature 1..21: note = synthetic
  source 1..21: mol_type = other DNA
atctattacagtgggaccacc

SEQ ID NO: 342 - protein, 7 aa, synthetic construct
  REGION 1..7: note = synthetic
IYYSGTT

SEQ ID NO: 343 - DNA, 42 bp, synthetic construct
  misc_feature 1..42: note = synthetic
  source 1..42: mol_type = other DNA
gcgagagagtcgtataatccctcgccgcgatattttgaccac

SEQ ID NO: 344 - protein, 14 aa, synthetic construct
  REGION 1..14: note = synthetic
ARESYNPSPRYFDH

SEQ ID NO: 345 - DNA, 375 bp, synthetic construct
  misc_feature 1..375: note = synthetic
  source 1..375: mol_type = other DNA
caggtgcagctggtggagtctgggggaggcgtggtccagcctgggaggtccctgagactctcctgtgcagcgtctggattcagcttcagtagttatggcatgcactgggtccgccaggctccaggcaaggggctggagtggatggcagttatatggtatgctggaagtaataaattctatgcagactccgtgaagggccgattcaccatctccagagacaattccaagaacacgctgtatctgcaaatgaacagcctgacagccgaggacacggctgtatattactgtgcgagagggtcgagtctagcagctccagacctctacaagtacggaatggacgtctggggccaggggaccacggtcaccgtctcctca

SEQ ID NO: 346 - protein, 125 aa, synthetic construct
  REGION 1..125: note = synthetic
QVQLVESGGGVVQPGRSLRLSCAASGFSFSSYGMHWVRQAPGKGLEWMAVIWYAGSNKFYADSVKGRFTISRDNSKNTLYLQMNSLTAEDTAVYYCARGSSLAAPDLYKYGMDVWGQGTTVTVSS

SEQ ID NO: 347 - DNA, 24 bp, synthetic construct
  misc_feature 1..24: note = synthetic
  source 1..24: mol_type = other DNA
ggattcagcttcagtagttatggc

SEQ ID NO: 348 - protein, 8 aa, synthetic construct
  REGION 1..8: note = synthetic
GFSFSSYG

SEQ ID NO: 349 - DNA, 24 bp, synthetic construct
  misc_feature 1..24: note = synthetic
  source 1..24: mol_type = other DNA
atatggtatgctggaagtaataaa

SEQ ID NO: 350 - protein, 8 aa, synthetic construct
  REGION 1..8: note = synthetic
IWYAGSNK

SEQ ID NO: 351 - DNA, 54 bp, synthetic construct
  misc_feature 1..54: note = synthetic
  source 1..54: mol_type = other DNA
gcgagagggtcgagtctagcagctccagacctctacaagtacggaatggacgtc

SEQ ID NO: 352 - protein, 18 aa, synthetic construct
  REGION 1..18: note = synthetic
ARGSSLAAPDLYKYGMDV

SEQ ID NO: 353 - DNA, 351 bp, synthetic construct
  misc_feature 1..351: note = synthetic
  source 1..351: mol_type = other DNA
caggtgcagctgcaggagtcgggcccaggactggtgaagccttcggagaccctgtccctcacctgtactatctctggtggctccatcagtaattccttcttgacctggatccgacagcccccagggaagggactggagtggattggatatatctatcaccggggaaacactgattccaatccctccctcaagagtcgagtcaccatctcaacagacccgtccaagaatcagttctccctgaccctgcactctgtgaccgccgcagactcggccatatattactgtgcgcggggacaatttatggagtggtttgacttctggggccagggaaccctggtcaccgtctcctca

SEQ ID NO: 354 - protein, 117 aa, synthetic construct
  REGION 1..117: note = synthetic
QVQLQESGPGLVKPSETLSLTCTISGGSISNSFLTWIRQPPGKGLEWIGYIYHRGNTDSNPSLKSRVTISTDPSKNQFSLTLHSVTAADSAIYYCARGQFMEWFDFWGQGTLVTVSS

SEQ ID NO: 355 - DNA, 24 bp, synthetic construct
  misc_feature 1..24: note = synthetic
  source 1..24: mol_type = other DNA
ggtggctccatcagtaattccttc

SEQ ID NO: 356 - protein, 8 aa, synthetic construct
  REGION 1..8: note = synthetic
GGSISNSF

SEQ ID NO: 357 - DNA, 21 bp, synthetic construct
  misc_feature 1..21: note = synthetic
  source 1..21: mol_type = other DNA
atctatcaccggggaaacact

SEQ ID NO: 358 - protein, 7 aa, synthetic construct
  REGION 1..7: note = synthetic
IYHRGNT

SEQ ID NO: 359 - DNA, 33 bp, synthetic construct
  misc_feature 1..33: note = synthetic
  source 1..33: mol_type = other DNA
gcgcggggacaatttatggagtggtttgacttc

SEQ ID NO: 360 - protein, 11 aa, synthetic construct
  REGION 1..11: note = synthetic
ARGQFMEWFDF

SEQ ID NO: 361 - DNA, 375 bp, synthetic construct
  misc_feature 1..375: note = synthetic
  source 1..375: mol_type = other DNA
caggtgcagctggtggagtctgggggaggcgtggtccagcctgggaggtccctgagagtctcctgtgaagcgtctggattcaccctcagtagttatggcatgaactgggtccgccaggctccaggcaaggggctggagtgggtggcagttatatggtatgatggaagtaataaatactattcagactccgtgaagggccgattcaccatctccagagacaattccaagaacacgctgtatctgcaaatgaacggcctgagagacgatgacacggctgtgtattactgtgcgagaggggagcagctcggctctcatgtctattattactatggaatggacgtctggggccaagggaccacggtcaccgtctcctca

SEQ ID NO: 362 - protein, 125 aa, synthetic construct
  REGION 1..125: note = synthetic
QVQLVESGGGVVQPGRSLRVSCEASGFTLSSYGMNWVRQAPGKGLEWVAVIWYDGSNKYYSDSVKGRFTISRDNSKNTLYLQMNGLRDDDTAVYYCARGEQLGSHVYYYYGMDVWGQGTTVTVSS

SEQ ID NO: 363 - DNA, 24 bp, synthetic construct
  misc_feature 1..24: note = synthetic
  source 1..24: mol_type = other DNA
ggattcaccctcagtagttatggc

SEQ ID NO: 364 - protein, 8 aa, synthetic construct
  REGION 1..8: note = synthetic
GFTLSSYG

SEQ ID NO: 365 - DNA, 24 bp, synthetic construct
  misc_feature 1..24: note = synthetic
  source 1..24: mol_type = other DNA
atatggtatgatggaagtaataaa

SEQ ID NO: 366 - protein, 8 aa, synthetic construct
  REGION 1..8: note = synthetic
IWYDGSNK

SEQ ID NO: 367 - DNA, 54 bp, synthetic construct
  misc_feature 1..54: note = synthetic
  source 1..54: mol_type = other DNA
gcgagaggggagcagctcggctctcatgtctattattactatggaatggacgtc

SEQ ID NO: 368 - protein, 18 aa, synthetic construct
  REGION 1..18: note = synthetic
ARGEQLGSHVYYYYGMDV

SEQ ID NO: 369 - DNA, 375 bp, synthetic construct
  misc_feature 1..375: note = synthetic
  source 1..375: mol_type = other DNA
caggtgcagctggtggagtctgggggaggcgtggtccagcctgggaagtccctgagactctcctgtgcagcgtctggattcaccttcagtaactatgtcatgcactgggtccgccagactccaggcaaggggctggagtgggtggcgattattttatttcctggaagtaataaatactatgtagactccgtgcagggccgattcaccatctccagagacaattccaagaacacgctgtctctgcaaatgaacagcctgagagccgaagacacggctgtatattactgtgcgaggggctcgagtttgacagctcttgactactactactacggtctggacgtctggggccaagggaccacggtcaccgtctcctca

SEQ ID NO: 370 - protein, 125 aa, synthetic construct
  REGION 1..125: note = synthetic
QVQLVESGGGVVQPGKSLRLSCAASGFTFSNYVMHWVRQTPGKGLEWVAIILFPGSNKYYVDSVQGRFTISRDNSKNTLSLQMNSLRAEDTAVYYCARGSSLTALDYYYYGLDVWGQGTTVTVSS

SEQ ID NO: 371 - DNA, 24 bp, synthetic construct
  misc_feature 1..24: note = synthetic
  source 1..24: mol_type = other DNA
ggattcaccttcagtaactatgtc

SEQ ID NO: 372 - protein, 8 aa, synthetic construct
  REGION 1..8: note = synthetic
GFTFSNYV

SEQ ID NO: 373 - DNA, 24 bp, synthetic construct
  misc_feature 1..24: note = synthetic
  source 1..24: mol_type = other DNA
attttatttcctggaagtaataaa

SEQ ID NO: 374 - protein, 8 aa, synthetic construct
  REGION 1..8: note = synthetic
ILFPGSNK

SEQ ID NO: 375 - DNA, 54 bp, synthetic construct
  misc_feature 1..54: note = synthetic
  source 1..54: mol_type = other DNA
gcgaggggctcgagtttgacagctcttgactactactactacggtctggacgtc

SEQ ID NO: 376 - protein, 18 aa, synthetic construct
  REGION 1..18: note = synthetic
ARGSSLTALDYYYYGLDV

SEQ ID NO: 377 - DNA, 375 bp, synthetic construct
  misc_feature 1..375: note = synthetic
  source 1..375: mol_type = other DNA
caggtgcagctggtggagtctgggggaggcgtggtccagcctgggaggtccctgagactctcctgtgcagcgtctggattcaccttcagtaactatgtcatgcactgggtccgccaggctccaggcaaggggctggagtgggtggcaattatatggtatgatggaactaatgaagactatgcagactccgtgaaggtccgattcaccatctccagagacatttccaagaacacgctgtatctgcaaatgaacagcctgagagccgaggacacggctgtatattactgtgcgagagattggtttgattgtagtagtaccagctgctataggtacttcgatctctggggccgtggcaccctggtcactgtctcctca

SEQ ID NO: 378 - protein, 125 aa, synthetic construct
  REGION 1..125: note = synthetic
QVQLVESGGGVVQPGRSLRLSCAASGFTFSNYVMHWVRQAPGKGLEWVAIIWYDGTNEDYADSVKVRFTISRDISKNTLYLQMNSLRAEDTAVYYCARDWFDCSSTSCYRYFDLWGRGTLVTVSS

SEQ ID NO: 379 - DNA, 24 bp, synthetic construct
  misc_feature 1..24: note = synthetic
  source 1..24: mol_type = other DNA
ggattcaccttcagtaactatgtc

SEQ ID NO: 380 - protein, 8 aa, synthetic construct
  REGION 1..8: note = synthetic
GFTFSNYV

SEQ ID NO: 381 - DNA, 24 bp, synthetic construct
  misc_feature 1..24: note = synthetic
  source 1..24: mol_type = other DNA
atatggtatgatggaactaatgaa

SEQ ID NO: 382 - protein, 8 aa, synthetic construct
  REGION 1..8: note = synthetic
IWYDGTNE

SEQ ID NO: 383 - DNA, 54 bp, synthetic construct
  misc_feature 1..54: note = synthetic
  source 1..54: mol_type = other DNA
gcgagagattggtttgattgtagtagtaccagctgctataggtacttcgatctc

SEQ ID NO: 384 - protein, 18 aa, synthetic construct
  REGION 1..18: note = synthetic
ARDWFDCSSTSCYRYFDL

SEQ ID NO: 385 - DNA, 375 bp, synthetic construct
  misc_feature 1..375: note = synthetic
  source 1..375: mol_type = other DNA
caggtgcagctggtggagtctgggggaggcgtggtccagcctgggaggtccctgagactctcctgtgcagcgtctggattcaccttcagtaataataacatgcactgggtccgccaggctccaggcaaggggctggagtgggtggcagttatatggtatgatggaagtaataaagattatgtagactccgtgaagggccgattcaccatctccagagacaattccaagaacacgctgtatctgcaaatgaacagtttgagagccgaggatacggctgtgtattattgtgcgagatttgtagtagcgccagctacgtactcctactactacattatagacgtctggggccaagggaccacggtcaccgtctcctca

SEQ ID NO: 386 - protein, 125 aa, synthetic construct
  REGION 1..125: note = synthetic
QVQLVESGGGVVQPGRSLRLSCAASGFTFSNNNMHWVRQAPGKGLEWVAVIWYDGSNKDYVDSVKGRFTISRDNSKNTLYLQMNSLRAEDTAVYYCARFVVAPATYSYYYIIDVWGQGTTVTVSS

SEQ ID NO: 387 - DNA, 24 bp, synthetic construct
  misc_feature 1..24: note = synthetic
  source 1..24: mol_type = other DNA
ggattcaccttcagtaataataac

SEQ ID NO: 388 - protein, 8 aa, synthetic construct
  REGION 1..8: note = synthetic
GFTFSNNN

SEQ ID NO: 389 - DNA, 24 bp, synthetic construct
  misc_feature 1..24: note = synthetic
  source 1..24: mol_type = other DNA
atatggtatgatggaagtaataaa

SEQ ID NO: 390 - protein, 8 aa, synthetic construct
  REGION 1..8: note = synthetic
IWYDGSNK

SEQ ID NO: 391 - DNA, 54 bp, synthetic construct
  misc_feature 1..54: note = synthetic
  source 1..54: mol_type = other DNA
gcgagatttgtagtagcgccagctacgtactcctactactacattatagacgtc

SEQ ID NO: 392 - protein, 18 aa, synthetic construct
  REGION 1..18: note = synthetic
ARFVVAPATYSYYYIIDV

SEQ ID NO: 393 - DNA, 378 bp, synthetic construct
  misc_feature 1..378: note = synthetic
  source 1..378: mol_type = other DNA
caggtgcagctggtggagtctgggggaggcgtggtccagcctgggaggtccctgagactctcctgtgcagcctctggatttaccttcagtacctatggcatgcactgggtccgccaggctccaggcaaggggctggagtgggtggcagttatttcatatgatggaagaattaaatactatgaagactccgtgaagggccgattcatcatatccagagacaactccaagaacacactgtatctgcaagtgaacaccctgagagctgaggacacggctgtgtattactgtgcgaaagagaggagatattgtagtgatactaatacctgctctgatgtttttgatgtctggggccaggggacaatggtcaccgtctcttca

SEQ ID NO: 394 - protein, 126 aa, synthetic construct
  REGION 1..126: note = synthetic
QVQLVESGGGVVQPGRSLRLSCAASGFTFSTYGMHWVRQAPGKGLEWVAVISYDGRIKYYEDSVKGRFIISRDNSKNTLYLQVNTLRAEDTAVYYCAKERRYCSDTNTCSDVFDVWGQGTMVTVSS

SEQ ID NO: 395 - DNA, 24 bp, synthetic construct
  misc_feature 1..24: note = synthetic
  source 1..24: mol_type = other DNA
ggatttaccttcagtacctatggc

SEQ ID NO: 396 - protein, 8 aa, synthetic construct
  REGION 1..8: note = synthetic
GFTFSTYG

SEQ ID NO: 397 - DNA, 24 bp, synthetic construct
  misc_feature 1..24: note = synthetic
  source 1..24: mol_type = other DNA
atttcatatgatggaagaattaaa

SEQ ID NO: 398 - protein, 8 aa, synthetic construct
  REGION 1..8: note = synthetic
ISYDGRIK

SEQ ID NO: 399 - DNA, 57 bp, synthetic construct
  misc_feature 1..57: note = synthetic
  source 1..57: mol_type = other DNA
gcgaaagagaggagatattgtagtgatactaatacctgctctgatgtttttgatgtc

SEQ ID NO: 400 - protein, 19 aa, synthetic construct
  REGION 1..19: note = synthetic
AKERRYCSDTNTCSDVFDV

SEQ ID NO: 401 - DNA, 324 bp, synthetic construct
  misc_feature 1..324: note = synthetic
  source 1..324: mol_type = other DNA
gacatccagatgacccagtctccatcctccctgtctgcatctgtaggagacagagtcaccatcacttgccgggcaagtcagagcattagcagctatttaaattggtatcagcagaaaccagggaaagcccctaagctcctgatctatgctgcatccagtttgcaaagtggggtcccgtcaaggttcagtggcagtggatctgggacagatttcactctcaccatcagcagtctgcaacctgaagattttgcaacttactactgtcaacagagttacagtacccctccgatcaccttcggccaagggacacgactggagattaaa

SEQ ID NO: 402 - protein, 108 aa, synthetic construct
  REGION 1..108: note = synthetic
DIQMTQSPSSLSASVGDRVTITCRASQSISSYLNWYQQKPGKAPKLLIYAASSLQSGVPSRFSGSGSGTDFTLTISSLQPEDFATYYCQQSYSTPPITFGQGTRLEIK

SEQ ID NO: 403 - DNA, 18 bp, synthetic construct
  misc_feature 1..18: note = synthetic
  source 1..18: mol_type = other DNA
cagagcattagcagctat

SEQ ID NO: 404 - protein, 6 aa, synthetic construct
  REGION 1..6: note = synthetic
QSISSY

SEQ ID NO: 405-406 - skipped (2 entries)

SEQ ID NO: 407 - DNA, 30 bp, synthetic construct
  misc_feature 1..30: note = synthetic
  source 1..30: mol_type = other DNA
caacagagttacagtacccctccgatcacc

SEQ ID NO: 408 - protein, 10 aa, synthetic construct
  REGION 1..10: note = synthetic
QQSYSTPPIT

SEQ ID NO: 409 - protein, 194 aa, synthetic construct
  REGION 1..194: note = synthetic
MHRPRRRGTRPPPLALLAALLLAARGADAQRPTGGPGCGPGRLLLGTGTDARCCRVHTTRCCRDYPGEECCSEWDCMCVQPEFHCGDPCCTTCRHHPCPPGQGVQSQGKFSFGFQCIDCASGTFSGGHEGHCKPWTDCTQFGFLTVFPGNKTHNAVCVPGSPPAEPEQKLISEEDLGGEQKLISEEDLHHHHHH

SEQ ID NO: 410 - protein, 399 aa, synthetic construct
  REGION 1..399: note = synthetic
MHRPRRRGTRPPPLALLAALLLAARGADAQRPTGGPGCGPGRLLLGTGTDARCCRVHTTRCCRDYPGEECCSEWDCMCVQPEFHCGDPCCTTCRHHPCPPGQGVQSQGKFSFGFQCIDCASGTFSGGHEGHCKPWTDCTQFGFLTVFPGNKTHNAVCVPGSPPAEPEPRGPTIKPCPPCKCPAPNLLGGPSVFIFPPKIKDVLMISLSPIVTCVVVDVSEDDPDVQISWFVNNVEVHTAQTQTHREDYNSTLRVVSALPIQHQDWMSGKEFKCKVNNKDLPAPIERTISKPKGSVRAPQVYVLPPPEEEMTKKQVTLTCMVTDFMPEDIYVEWTNNGKTELNYKNTEPVLDSDGSYFMYSKLRVEKKNWVERNSYSCSVVHEGLHNHHTTKSFSRTPGK

SEQ ID NO: 411 - protein, 393 aa, synthetic construct
  REGION 1..393: note = synthetic
MHRPRRRGTRPPPLALLAALLLAARGADAQRPTGGPGCGPGRLLLGTGTDARCCRVHTTRCCRDYPGEECCSEWDCMCVQPEFHCGDPCCTTCRHHPCPPGQGVQSQGKFSFGFQCIDCASGTFSGGHEGHCKPWTDCTQFGFLTVFPGNKTHNAVCVPGSPPAEPDKTHTCPPCPAPELLGGPSVFLFPPKPKDTLMISRTPEVTCVVVDVSHEDPEVKFNWYVDGVEVHNAKTKPREEQYNSTYRVVSVLTVLHQDWLNGKEYKCKVSNKALPAPIEKTISKAKGQPREPQVYTLPPSRDELTKNQVSLTCLVKGFYPSDIAVEWESNGQPENNYKTTPPVLDSDGSFFLYSKLTVDKSRWQQGNVFSCSVMHEALHNHYTQKSLSLSPGK

SEQ ID NO: 412 - protein, 194 aa, synthetic construct
  REGION 1..194: note = synthetic
MHRPRRRGTRPPPLALLAALLLAARGADAQRPTGGPGCGPGRLLLGTGKDARCCRVHPTRCCRDYQGEECCSEWDCVCVQPEFHCGNPCCTTCQHHPCPSGQGVQPQGKFSFGFRCVDCALGTFSRGHDGHCKPWTDCTQFGFLTVFPGNKTHNAVCVPGSPPAEPEQKLISEEDLGGEQKLISEEDLHHHHHH

SEQ ID NO: 413 - protein, 241 aa, synthetic construct
  REGION 1..241: note = synthetic
MAQHGAMGAFRALCGLALLCALSLGQRPTGGPGCGPGRLLLGTGTDARCCRVHTTRCCRDYPGEECCSEWDCMCVQPEFHCGDPCCTTCRHHPCPPGQGVQSQGKFSFGFQCIDCASGTFSGGHEGHCKPWTDCTQFGFLTVFPGNKTHNAVCVPGSPPAEPLGWLTVVLLAVAACVLLLTSAQLGLHIWQLRSQCMWPRETQLLLEVPPSTEDARSCQFPEEERGERSAEEKGRLGDLWV